European Patent Specification EP 3 824 905 B1, published January 8, 2025. Title: METHOD AND COMPOSITIONS FOR CELLULAR IMMUNOTHERAPY. Applicant: Jensen, Michael Riddell, Stanley R. Hudecek, Michael. Application New Filing. The sequence listing filed with the application follows.

SEQUENCE LISTING (56 sequences)

SEQ ID NO: 1 - protein, 5 aa, Artificial Sequence
  Synthetic
  MISC_FEATURE (1)..(1): Xaa is glycine, cysteine or arginine
  MISC_FEATURE (4)..(4): Xaa is cysteine or threonine
XPPXP

SEQ ID NO: 2 - DNA, 66 bp, Artificial Sequence
  Synthetic
atgctgctgctggtgaccagcctgctgctgtgcgagctgccccaccccgcctttctgctgatcccc

SEQ ID NO: 3 - DNA, 735 bp, Artificial Sequence
  Synthetic
gacatccagatgacccagaccacctccagcctgagcgccagcctgggcgaccgggtgaccatcagctgccgggccagccaggacatcagcaagtacctgaactggtatcagcagaagcccgacggcaccgtcaagctgctgatctaccacaccagccggctgcacagcggcgtgcccagccggtttagcggcagcggctccggcaccgactacagcctgaccatctccaacctggaacaggaagatatcgccacctacttttgccagcagggcaacacactgccctacacctttggcggcggaacaaagctggaaatcaccggcagcacctccggcagcggcaagcctggcagcggcgagggcagcaccaagggcgaggtgaagctgcaggaaagcggccctggcctggtggcccccagccagagcctgagcgtgacctgcaccgtgagcggcgtgagcctgcccgactacggcgtgagctggatccggcagccccccaggaagggcctggaatggctgggcgtgatctggggcagcgagaccacctactacaacagcgccctgaagagccggctgaccatcatcaaggacaacagcaagagccaggtgttcctgaagatgaacagcctgcagaccgacgacaccgccatctactactgcgccaagcactactactacggcggcagctacgccatggactactggggccagggcaccagcgtgaccgtgagcagc

SEQ ID NO: 4 - DNA, 36 bp, Artificial Sequence
  Synthetic
gaatctaagtacggaccgccctgccccccttgccct

SEQ ID NO: 5 - DNA, 84 bp, Artificial Sequence
  Synthetic
atgttctgggtgctggtggtggtcggaggcgtgctggcctgctacagcctgctggtcaccgtggccttcatcatcttttgggtg

SEQ ID NO: 6 - DNA, 126 bp, Artificial Sequence
  Synthetic
aaacggggcagaaagaaactcctgtatatattcaaacaaccatttatgagaccagtacaaactactcaagaggaagatggctgtagctgccgatttccagaagaagaagaaggaggatgtgaactg

SEQ ID NO: 7 - DNA, 336 bp, Artificial Sequence
  Synthetic
cgggtgaagttcagcagaagcgccgacgcccctgcctaccagcagggccagaatcagctgtacaacgagctgaacctgggcagaagggaagagtacgacgtcctggataagcggagaggccgggaccctgagatgggcggcaagcctcggcggaagaacccccaggaaggcctgtataacgaactgcagaaagacaagatggccgaggcctacagcgagatcggcatgaagggcgagcggaggcggggcaagggccacgacggcctgtatcagggcctgtccaccgccaccaaggatacctacgacgccctgcacatgcaggccctgcccccaagg

SEQ ID NO: 8 - DNA, 72 bp, Artificial Sequence
  Synthetic
ctcgagggcggcggagagggcagaggaagtcttctaacatgcggtgacgtggaggagaatcccggccctagg

SEQ ID NO: 9 - DNA, 1074 bp, Artificial Sequence
  Synthetic
atgcttctcctggtgacaagccttctgctctgtgagttaccacacccagcattcctcctgatcccacgcaaagtgtgtaacggaataggtattggtgaatttaaagactcactctccataaatgctacgaatattaaacacttcaaaaactgcacctccatcagtggcgatctccacatcctgccggtggcatttaggggtgactccttcacacatactcctcctctggatccacaggaactggatattctgaaaaccgtaaaggaaatcacagggtttttgctgattcaggcttggcctgaaaacaggacggacctccatgcctttgagaacctagaaatcatacgcggcaggaccaagcaacatggtcagttttctcttgcagtcgtcagcctgaacataacatccttgggattacgctccctcaaggagataagtgatggagatgtgataatttcaggaaacaaaaatttgtgctatgcaaatacaataaactggaaaaaactgtttgggacctccggtcagaaaaccaaaattataagcaacagaggtgaaaacagctgcaaggccacaggccaggtctgccatgccttgtgctcccccgagggctgctggggcccggagcccagggactgcgtctcttgccggaatgtcagccgaggcagggaatgcgtggacaagtgcaaccttctggagggtgagccaagggagtttgtggagaactctgagtgcatacagtgccacccagagtgcctgcctcaggccatgaacatcacctgcacaggacggggaccagacaactgtatccagtgtgcccactacattgacggcccccactgcgtcaagacctgcccggcaggagtcatgggagaaaacaacaccctggtctggaagtacgcagacgccggccatgtgtgccacctgtgccatccaaactgcacctacggatgcactgggccaggtcttgaaggctgtccaacgaatgggcctaagatcccgtccatcgccactgggatggtgggggccctcctcttgctgctggtggtggccctggggatcggcctcttcatgtga

SEQ ID NO: 10 - DNA, 2529 bp, Artificial Sequence
  Synthetic
atgctgctgctggtgaccagcctgctgctgtgcgagctgccccaccccgcctttctgctgatccccgacatccagatgacccagaccacctccagcctgagcgccagcctgggcgaccgggtgaccatcagctgccgggccagccaggacatcagcaagtacctgaactggtatcagcagaagcccgacggcaccgtcaagctgctgatctaccacaccagccggctgcacagcggcgtgcccagccggtttagcggcagcggctccggcaccgactacagcctgaccatctccaacctggaacaggaagatatcgccacctacttttgccagcagggcaacacactgccctacacctttggcggcggaacaaagctggaaatcaccggcagcacctccggcagcggcaagcctggcagcggcgagggcagcaccaagggcgaggtgaagctgcaggaaagcggccctggcctggtggcccccagccagagcctgagcgtgacctgcaccgtgagcggcgtgagcctgcccgactacggcgtgagctggatccggcagccccccaggaagggcctggaatggctgggcgtgatctggggcagcgagaccacctactacaacagcgccctgaagagccggctgaccatcatcaaggacaacagcaagagccaggtgttcctgaagatgaacagcctgcagaccgacgacaccgccatctactactgcgccaagcactactactacggcggcagctacgccatggactactggggccagggcaccagcgtgaccgtgagcagcgagagcaagtacggaccgccctgccccccttgccctatgttctgggtgctggtggtggtcggaggcgtgctggcctgctacagcctgctggtcaccgtggccttcatcatcttttgggtgaaacggggcagaaagaaactcctgtatatattcaaacaaccatttatgagaccagtacaaactactcaagaggaagatggctgtagctgccgatttccagaagaagaagaaggaggatgtgaactgcgggtgaagttcagcagaagcgccgacgcccctgcctaccagcagggccagaatcagctgtacaacgagctgaacctgggcagaagggaagagtacgacgtcctggataagcggagaggccgggaccctgagatgggcggcaagcctcggcggaagaacccccaggaaggcctgtataacgaactgcagaaagacaagatggccgaggcctacagcgagatcggcatgaagggcgagcggaggcggggcaagggccacgacggcctgtatcagggcctgtccaccgccaccaaggatacctacgacgccctgcacatgcaggccctgcccccaaggctcgagggcggcggagagggcagaggaagtcttctaacatgcggtgacgtggaggagaatcccggccctaggatgcttctcctggtgacaagccttctgctctgtgagttaccacacccagcattcctcctgatcccacgcaaagtgtgtaacggaataggtattggtgaatttaaagactcactctccataaatgctacgaatattaaacacttcaaaaactgcacctccatcagtggcgatctccacatcctgccggtggcatttaggggtgactccttcacacatactcctcctctggatccacaggaactggatattctgaaaaccgtaaaggaaatcacagggtttttgctgattcaggcttggcctgaaaacaggacggacctccatgcctttgagaacctagaaatcatacgcggcaggaccaagcaacatggtcagttttctcttgcagtcgtcagcctgaacataacatccttgggattacgctccctcaaggagataagtgatggagatgtgataatttcaggaaacaaaaatttgtgctatgcaaatacaataaactggaaaaaactgtttgggacctccggtcagaaaaccaaaattataagcaacagaggtgaaaacagctgcaaggccacaggccaggtctgccatgccttgtgctcccccgagggctgctggggcccggagcccagggactgcgtctcttgccggaatgtcagccgaggcagggaatgcgtggacaagtgcaaccttctggagggtgagccaagggagtttgtggagaactctgagtgcatacagtgccacccagagtgcctgcctcaggccatgaacatcacctgcacaggacggggaccagacaactgtatccagtgtgcccactacattgacggcccccactgcgtcaagacctgcccggcaggagtcatgggagaaaacaacaccctggtctggaagtacgcagacgccggccatgtgtgccacctgtgccatccaaactgcacctacggatgcactgggccaggtcttgaaggctgtccaacgaatgggcctaagatcccgtccatcgccactgggatggtgggggccctcctcttgctgctggtggtggccctggggatcggcctcttcatgtga

SEQ ID NO: 11 - protein, 841 aa, Artificial Sequence
  Synthetic
MLLLVTSLLLCELPHPAFLLIPDIQMTQTTSSLSASLGDRVTISCRASQDISKYLNWYQQKPDGTVKLLIYHTSRLHSGVPSRFSGSGSGTDYSLTISNLEQEDIATYFCQQGNTLPYTFGGGTKLEITGSTSGSGKPGSGEGSTKGEVKLQESGPGLVAPSQSLSVTCTVSGVSLPDYGVSWIRQPPRKGLEWLGVIWGSETTYYNSALKSRLTIIKDNSKSQVFLKMNSLQTDDTAIYYCAKHYYYGGSYAMDYWGQGTSVTVSSESKYGPPCPPCPMFWVLVVVGGVLACYSLLVTVAFIIFWVKRGRKKLLYIFKQPFMRPVQTTQEEDGCSCRFEEEEGGCELRVKFSRSADAPAYQQGQNQLYNELNLGRREEYDVLDKRRGRDPEMGGKPRRKNPQEGLYNELQKDKMAEAYSEIGMKGERRRGKGHDGLYQGLSTATKDTYDALHMQALPPRLEGGGEGRGSLLTCGDVEENPGPRMLLLVTSLLLCELPHPAFLLIPRKVCNGIGIGEFKDSLSINATNIKHFKNCTSISGDLHILPVAFRGDSFTHTPPLDPQELDILKTVKEITGFLLIQAWPENRTDLHAFENLEIIRGRTKQHGQFSLAVVSLNITSLGLRSLKEISDGDVIISGNKNLCYANTINWKKLFGTSGQKTKIISNRGENSCKATGQVCHALCSPEGCWGPEPRDCVSCRNVSRGRECVDKCNLLEGEPREFVENSECIQCHPECLPQAMNITCTGRGPDNCIQCAHYIDGPHCVKTCPAGVMGENNTLVWKYADAGHVCHLCHPNCTYGCTGPGLEGCPTNGPKIPSIATGMVGALLLLLVVALGIGLFM

SEQ ID NO: 12 - protein, 15 aa, Artificial Sequence
  Synthetic
GGGGSGGGGSGGGGS

SEQ ID NO: 13 - protein, 327 aa, Homo sapiens
ASTKGPSVFPLAPCSRSTSESTAALGCLVKDYFPEPVTVSWNSGALTSGVHTFPAVLQSSGLYSLSSVVTVPSSSLGTKTYTCNVDHKPSNTKVDKRVESKYGPPCPSCPAPEFLGGPSVFLFPPKPKDTLMISRTPEVTCVVVDVSQEDPEVQFNWYVDGVEVHNAKTKPREEQFNSTYRVVSVLTVLHQDWLNGKEYKCKVSNKGLPSSIEKTISKAKGQPREPQVYTLPPSQEEMTKNQVSLTCLVKGFYPSDIAVEWESNGQPENNYKTTPPVLDSDGSFFLYSRLTVDKSRWQEGNVFSCSVMHEALHNHYTQKSLSLSLGK

SEQ ID NO: 14 - protein, 220 aa, Homo sapiens
MLRLLLALNLFPSIQVTGNKILVKQSPMLVAYDNAVNLSCKYSYNLFSREFRASLHKGLDSAVEVCVVYGNYSQQLQVYSKTGFNCDGKLGNESVTFYLQNLYVNQTDIYFCKIEVMYPPPYLDNEKSNGTIIHVKGKHLCPSPLFPGPSKPFWVLVVVGGVLACYSLLVTVAFIIFWVRSKRSRLLHSDYMNMTPRRPGPTRKHYQPYAPPRDFAAYRS

SEQ ID NO: 15 - protein, 255 aa, Homo sapiens
MGNSCYNIVATLLLVLNFERTRSLQDPCSNCPAGTFCDNNRNQICSPCPPNSFSSAGGQRTCDICRQCKGVFRTRKECSSTSNAECDCTPGFHCLGAGCSMCEQDCKQGQELTKKGCKDCCFGTFNDQKRGICRPWTNCSLDGKSVLVNGTKERDVVCGPSPADLSPGASSVTPPAPAREPGHSPQIISFFLALTSTALLFLLFFLTLRFSVVKRGRKKLLYIFKQPFMRPVQTTQEEDGCSCRFPEEEEGGCEL

SEQ ID NO: 16 - protein, 164 aa, Homo sapiens
MKWKALFTAAILQAQLPITEAQSFGLLDPKLCYLLDGILFIYGVILTALFLRVKFSRSADAPAYQQGQNQLYNELNLGRREEYDVLDKRRGRDPEMGGKPQRRKNPQEGLYNELQKDKMAEAYSEIGMKGERRRGKGHDGLYQGLSTATKDTYDALHMQALPPR

SEQ ID NO: 17 - protein, 15 aa, Homo sapiens
EPKSCDKTHTCPPCP

SEQ ID NO: 18 - protein, 12 aa, Homo sapiens
ERKCCVECPPCP

SEQ ID NO: 19 - protein, 61 aa, Homo sapiens
ELKTPLGDTHTCPRCPEPKSCDTPPPCPRCPEPKSCDTPPPCPRCPEPKSCDTPPPCPRCP

SEQ ID NO: 20 - protein, 12 aa, Homo sapiens
ESKYGPPCPSCP

SEQ ID NO: 21 - protein, 12 aa, Artificial Sequence
  Synthetic
ESKYGPPCPPCP

SEQ ID NO: 22 - DNA, 26 bp, Artificial Sequence
  Primer
atcaaaagaatagaccgagatagggt

SEQ ID NO: 23 - DNA, 26 bp, Artificial Sequence
  Primer
ccgtacctttaagaccaatgacttac

SEQ ID NO: 24 - DNA, 18 bp, Artificial Sequence
  Primer
ttgagagttttcgccccg

SEQ ID NO: 25 - DNA, 24 bp, Artificial Sequence
  Primer
aatagacagatcgctgagataggt

SEQ ID NO: 26 - DNA, 18 bp, Artificial Sequence
  Primer
caggtatccggtaagcgg

SEQ ID NO: 27 - DNA, 19 bp, Artificial Sequence
  Primer
cgaccagcaaccatagtcc

SEQ ID NO: 28 - DNA, 18 bp, Artificial Sequence
  Primer
tagcggtttgactcacgg

SEQ ID NO: 29 - DNA, 20 bp, Artificial Sequence
  Primer
gcagggagctagaacgattc

SEQ ID NO: 30 - DNA, 22 bp, Artificial Sequence
  Primer
attgtctggtatagtgcagcag

SEQ ID NO: 31 - DNA, 16 bp, Artificial Sequence
  Primer
tcgcaacgggtttgcc

SEQ ID NO: 32 - DNA, 21 bp, Artificial Sequence
  Primer
aggaagatatcgccacctact

SEQ ID NO: 33 - DNA, 20 bp, Artificial Sequence
  Primer
cgggtgaagttcagcagaag

SEQ ID NO: 34 - DNA, 20 bp, Artificial Sequence
  Primer
actgtgtttgctgacgcaac

SEQ ID NO: 35 - DNA, 20 bp, Artificial Sequence
  Primer
atgcttctcctggtgacaag

SEQ ID NO: 36 - protein, 18 aa, Artificial Sequence
  Synthetic
GSTSGSGKPGSGEGSTKG

SEQ ID NO: 37 - DNA, 10051 bp, Artificial Sequence
  Synthetic
gttagaccagatctgagcctgggagctctctggctaactagggaacccactgcttaagcctcaataaagcttgccttgagtgcttcaagtagtgtgtgcccgtctgttgtgtgactctggtaactagagatccctcagacccttttagtcagtgtggaaaatctctagcagtggcgcccgaacagggacttgaaagcgaaagggaaaccagaggagctctctcgacgcaggactcggcttgctgaagcgcgcacggcaagaggcgaggggcggcgactggtgagtacgccaaaaattttgactagcggaggctagaaggagagagatgggtgcgagagcgtcagtattaagcgggggagaattagatcgatgggaaaaaattcggttaaggccagggggaaagaaaaaatataaattaaaacatatagtatgggcaagcagggagctagaacgattcgcagttaatcctggcctgttagaaacatcagaaggctgtagacaaatactgggacagctacaaccatcccttcagacaggatcagaagaacttagatcattatataatacagtagcaaccctctattgtgtgcatcaaaggatagagataaaagacaccaaggaagctttagacaagatagaggaagagcaaaacaaaagtaagaaaaaagcacagcaagcagcagctgacacaggacacagcaatcaggtcagccaaaattaccctatagtgcagaacatccaggggcaaatggtacatcaggccatatcacctagaactttaaatgcatgggtaaaagtagtagaagagaaggctttcagcccagaagtgatacccatgttttcagcattatcagaaggagccaccccacaagatttaaacaccatgctaaacacagtggggggacatcaagcagccatgcaaatgttaaaagagaccatcaatgaggaagctgcaggcaaagagaagagtggtgcagagagaaaaaagagcagtgggaataggagctttgttccttgggttcttgggagcagcaggaagcactatgggcgcagcgtcaatgacgctgacggtacaggccagacaattattgtctggtatagtgcagcagcagaacaatttgctgagggctattgaggcgcaacagcatctgttgcaactcacagtctggggcatcaagcagctccaggcaagaatcctggctgtggaaagatacctaaaggatcaacagctcctggggatttggggttgctctggaaaactcatttgcaccactgctgtgccttggatctacaaatggcagtattcatccacaattttaaaagaaaaggggggattggggggtacagtgcaggggaaagaatagtagacataatagcaacagacatacaaactaaagaattacaaaaacaaattacaaaaattcaaaattttcgggtttattacagggacagcagagatccagtttggggatcaattgcatgaagaatctgcttagggttaggcgttttgcgctgcttcgcgaggatctgcgatcgctccggtgcccgtcagtgggcagagcgcacatcgcccacagtccccgagaagttggggggaggggtcggcaattgaaccggtgcctagagaaggtggcgcggggtaaactgggaaagtgatgtcgtgtactggctccgcctttttcccgagggtgggggagaaccgtatataagtgcagtagtcgccgtgaacgttctttttcgcaacgggtttgccgccagaacacagctgaagcttcgaggggctcgcatctctccttcacgcgcccgccgccctacctgaggccgccatccacgccggttgagtcgcgttctgccgcctcccgcctgtggtgcctcctgaactgcgtccgccgtctaggtaagtttaaagctcaggtcgagaccgggcctttgtccggcgctcccttggagcctacctagactcagccggctctccacgctttgcctgaccctgcttgctcaactctacgtctttgtttcgttttctgttctgcgccgttacagatccaagctgtgaccggcgcctacggctagcgaattcctcgaggccaccatgctgctgctggtgacaagcctgctgctgtgcgagctgccccaccccgcctttctgctgatcccccaggaacagctcgtcgaaagcggcggcagactggtgacacctggcggcagcctgaccctgagctgcaaggccagcggcttcgacttcagcgcctactacatgagctgggtccgccaggcccctggcaagggactggaatggatcgccaccatctaccccagcagcggcaagacctactacgccacctgggtgaacggacggttcaccatctccagcgacaacgcccagaacaccgtggacctgcagatgaacagcctgacagccgccgaccgggccacctacttttgcgccagagacagctacgccgacgacggcgccctgttcaacatctggggccctggcaccctggtgacaatctctagcggcggaggcggatctggtggcggaggaagtggcggcggaggatctgagctggtgctgacccagagcccctctgtgtctgctgccctgggaagccctgccaagatcacctgtaccctgagcagcgcccacaagaccgacaccatcgactggtatcagcagctgcagggcgaggcccccagatacctgatgcaggtgcagagcgacggcagctacaccaagaggccaggcgtgcccgaccggttcagcggatctagctctggcgccgaccgctacctgatcatccccagcgtgcaggccgatgacgaggccgattactactgtggcgccgactacatcggcggctacgtgttcggcggaggcacccagctgaccgtgaccggcgagtctaagtacggaccgccctgccccccttgccctgcccccgagttcctgggcggacccagcgtgttcctgttcccccccaagcccaaggacaccctgatgatcagccggacccccgaggtgacctgcgtggtggtggacgtgagccaggaagatcccgaggtccagttcaattggtacgtggacggcgtggaagtgcacaacgccaagaccaagcccagagaggaacagttcaacagcacctaccgggtggtgtctgtgctgaccgtgctgcaccaggactggctgaacggcaaagaatacaagtgcaaggtgtccaacaagggcctgcccagcagcatcgaaaagaccatcagcaaggccaagggccagcctcgcgagccccaggtgtacaccctgcctccctcccaggaagagatgaccaagaaccaggtgtccctgacctgcctggtgaagggcttctaccccagcgacatcgccgtggagtgggagagcaacggccagcctgagaacaactacaagaccacccctcccgtgctggacagcgacggcagcttcttcctgtacagccggctgaccgtggacaagagccggtggcaggaaggcaacgtctttagctgcagcgtgatgcacgaggccctgcacaaccactacacccagaagagcctgagcctgtccctgggcaagatgttctgggtgctggtggtggtgggcggggtgctggcctgctacagcctgctggtgacagtggccttcatcatcttttgggtgaaacggggcagaaagaaactcctgtatatattcaaacaaccatttatgagaccagtacaaactactcaagaggaagatggctgtagctgccgatttccagaagaagaagaaggaggatgtgaactgcgggtgaagttcagcagaagcgccgacgcccctgcctaccagcagggccagaatcagctgtacaacgagctgaacctgggcagaagggaagagtacgacgtcctggataagcggagaggccgggaccctgagatgggcggcaagcctcggcggaagaacccccaggaaggcctgtataacgaactgcagaaagacaagatggccgaggcctacagcgagatcggcatgaagggcgagcggaggcggggcaagggccacgacggcctgtatcagggcctgtccaccgccaccaaggatacctacgacgccctgcacatgcaggccctgcccccaaggctcgagggcggcggagagggcagaggaagtcttctaacatgcggtgacgtggaggagaatcccggccctaggatgcttctcctggtgacaagccttctgctctgtgagttaccacacccagcattcctcctgatcccacgcaaagtgtgtaacggaataggtattggtgaatttaaagactcactctccataaatgctacgaatattaaacacttcaaaaactgcacctccatcagtggcgatctccacatcctgccggtggcatttaggggtgactccttcacacatactcctcctctggatccacaggaactggatattctgaaaaccgtaaaggaaatcacagggtttttgctgattcaggcttggcctgaaaacaggacggacctccatgcctttgagaacctagaaatcatacgcggcaggaccaagcaacatggtcagttttctcttgcagtcgtcagcctgaacataacatccttgggattacgctccctcaaggagataagtgatggagatgtgataatttcaggaaacaaaaatttgtgctatgcaaatacaataaactggaaaaaactgtttgggacctccggtcagaaaaccaaaattataagcaacagaggtgaaaacagctgcaaggccacaggccaggtctgccatgccttgtgctcccccgagggctgctggggcccggagcccagggactgcgtctcttgccggaatgtcagccgaggcagggaatgcgtggacaagtgcaaccttctggagggtgagccaagggagtttgtggagaactctgagtgcatacagtgccacccagagtgcctgcctcaggccatgaacatcacctgcacaggacggggaccagacaactgtatccagtgtgcccactacattgacggcccccactgcgtcaagacctgcccggcaggagtcatgggagaaaacaacaccctggtctggaagtacgcagacgccggccatgtgtgccacctgtgccatccaaactgcacctacggatgcactgggccaggtcttgaaggctgtccaacgaatgggcctaagatcccgtccatcgccactgggatggtgggggccctcctcttgctgctggtggtggccctggggatcggcctcttcatgtgagcggccgctctagacccgggctgcaggaattcgatatcaagcttatcgataatcaacctctggattacaaaatttgtgaaagattgactggtattcttaactatgttgctccttttacgctatgtggatacgctgctttaatgcctttgtatcatgctattgcttcccgtatggctttcattttctcctccttgtataaatcctggttgctgtctctttatgaggagttgtggcccgttgtcaggcaacgtggcgtggtgtgcactgtgtttgctgacgcaacccccactggttggggcattgccaccacctgtcagctcctttccgggactttcgctttccccctccctattgccacggcggaactcatcgccgcctgccttgcccgctgctggacaggggctcggctgttgggcactgacaattccgtggtgttgtcggggaaatcatcgtcctttccttggctgctcgcctgtgttgccacctggattctgcgcgggacgtccttctgctacgtcccttcggccctcaatccagcggaccttccttcccgcggcctgctgccggctctgcggcctcttccgcgtcttcgccttcgccctcagacgagtcggatctccctttgggccgcctccccgcatcgataccgtcgactagccgtacctttaagaccaatgacttacaaggcagctgtagatcttagccactttttaaaagaaaaggggggactggaagggctaattcactcccaaagaagacaagatctgctttttgcctgtactgggtctctctggttagaccagatctgagcctgggagctctctggctaactagggaacccactgcttaagcctcaataaagcttgccttgagtgcttcaagtagtgtgtgcccgtctgttgtgtgactctggtaactagagatccctcagacccttttagtcagtgtggaaaatctctagcagaattcgatatcaagcttatcgataccgtcgacctcgagggggggcccggtacccaattcgccctatagtgagtcgtattacaattcactggccgtcgttttacaacgtcgtgactgggaaaaccctggcgttacccaacttaatcgccttgcagcacatccccctttcgccagctggcgtaatagcgaagaggcccgcaccgatcgcccttcccaacagttgcgcagcctgaatggcgaatggaaattgtaagcgttaatattttgttaaaattcgcgttaaatttttgttaaatcagctcattttttaaccaataggccgaaatcggcaaaatcccttataaatcaaaagaatagaccgagatagggttgagtgttgttccagtttggaacaagagtccactattaaagaacgtggactccaacgtcaaagggcgaaaaaccgtctatcagggcgatggcccactacgtgaaccatcaccctaatcaagttttttggggtcgaggtgccgtaaagcactaaatcggaaccctaaagggagcccccgatttagagcttgacggggaaagccggcgaacgtggcgagaaaggaagggaagaaagcgaaaggagcgggcgctagggcgctggcaagtgtagcggtcacgctgcgcgtaaccaccacacccgccgcgcttaatgcgccgctacagggcgcgtcaggtggcacttttcggggaaatgtgcgcggaacccctatttgtttatttttctaaatacattcaaatatgtatccgctcatgagacaataaccctgataaatgcttcaataatattgaaaaaggaagagtatgagtattcaacatttccgtgtcgcccttattcccttttttgcggcattttgccttcctgtttttgctcacccagaaacgctggtgaaagtaaaagatgctgaagatcagttgggtgcacgagtgggttacatcgaactggatctcaacagcggtaagatccttgagagttttcgccccgaagaacgttttccaatgatgagcacttttaaagttctgctatgtggcgcggtattatcccgtattgacgccgggcaagagcaactcggtcgccgcatacactattctcagaatgacttggttgagtactcaccagtcacagaaaagcatcttacggatggcatgacagtaagagaattatgcagtgctgccataaccatgagtgataacactgcggccaacttacttctgacaacgatcggaggaccgaaggagctaaccgcttttttgcacaacatgggggatcatgtaactcgccttgatcgttgggaaccggagctgaatgaagccataccaaacgacgagcgtgacaccacgatgcctgtagcaatggcaacaacgttgcgcaaactattaactggcgaactacttactctagcttcccggcaacaattaatagactggatggaggcggataaagttgcaggaccacttctgcgctcggcccttccggctggctggtttattgctgataaatctggagccggtgagcgtgggtctcgcggtatcattgcagcactggggccagatggtaagccctcccgtatcgtagttatctacacgacggggagtcaggcaactatggatgaacgaaatagacagatcgctgagataggtgcctcactgattaagcattggtaactgtcagaccaagtttactcatatatactttagattgatttaaaacttcatttttaatttaaaaggatctaggtgaagatcctttttgataatctcatgaccaaaatcccttaacgtgagttttcgttccactgagcgtcagaccccgtagaaaagatcaaaggatcttcttgagatcctttttttctgcgcgtaatctgctgcttgcaaacaaaaaaaccaccgctaccagcggtggtttgtttgccggatcaagagctaccaactctttttccgaaggtaactggcttcagcagagcgcagataccaaatactgttcttctagtgtagccgtagttaggccaccacttcaagaactctgtagcaccgcctacatacctcgctctgctaatcctgttaccagtggctgctgccagtggcgataagtcgtgtcttaccgggttggactcaagacgatagttaccggataaggcgcagcggtcgggctgaacggggggttcgtgcacacagcccagcttggagcgaacgacctacaccgaactgagatacctacagcgtgagctatgagaaagcgccacgcttcccgaagggagaaaggcggacaggtatccggtaagcggcagggtcggaacaggagagcgcacgagggagcttccagggggaaacgcctggtatctttatagtcctgtcgggtttcgccacctctgacttgagcgtcgatttttgtgatgctcgtcaggggggcggagcctatggaaaaacgccagcaacgcggcctttttacggttcctggccttttgctggccttttgctcacatgttctttcctgcgttatcccctgattctgtggataaccgtattaccgcctttgagtgagctgataccgctcgccgcagccgaacgaccgagcgcagcgagtcagtgagcgaggaagcggaagagcgcccaatacgcaaaccgcctctccccgcgcgttggccgattcattaatgcagctggcacgacaggtttcccgactggaaagcgggcagtgagcgcaacgcaattaatgtgagttagctcactcattaggcaccccaggctttacactttatgcttccggctcgtatgttgtgtggaattgtgagcggataacaatttcacacaggaaacagctatgaccatgattacgccaagctcgaaattaaccctcactaaagggaacaaaagctggagctccaccgcggtggcggcctcgaggtcgagatccggtcgaccagcaaccatagtcccgcccctaactccgcccatcccgcccctaactccgcccagttccgcccattctccgccccatggctgactaattttttttatttatgcagaggccgaggccgcctcggcctctgagctattccagaagtagtgaggaggcttttttggaggcctaggcttttgcaaaaagcttcgacggtatcgattggctcatgtccaacattaccgccatgttgacattgattattgactagttattaatagtaatcaattacggggtcattagttcatagcccatatatggagttccgcgttacataacttacggtaaatggcccgcctggctgaccgcccaacgacccccgcccattgacgtcaataatgacgtatgttcccatagtaacgccaatagggactttccattgacgtcaatgggtggagtatttacggtaaactgcccacttggcagtacatcaagtgtatcatatgccaagtacgccccctattgacgtcaatgacggtaaatggcccgcctggcattatgcccagtacatgaccttatgggactttcctacttggcagtacatctacgtattagtcatcgctattaccatggtgatgcggttttggcagtacatcaatgggcgtggatagcggtttgactcacggggatttccaagtctccaccccattgacgtcaatgggagtttgttttggcaccaaaatcaacgggactttccaaaatgtcgtaacaactccgccccattgacgcaaatgggcggtaggcgtgtacggaattcggagtggcgagccctcagatcctgcatataagcagctgctttttgcctgtactgggtctctctg

SEQ ID NO: 38 - protein, 1062 aa, Artificial Sequence
  Synthetic
MLLLVTSLLLCELPHPAFLLIPQEQLVESGGRLVTPGGSLTLSCKASGFDFSAYYMSWVRQAPGKGLEWIATIYPSSGKTYYATWVNGRFTISSDNAQNTVDLQMNSLTAADRATYFCARDSYADDGALFNIWGPGTLVTISSGGGGSGGGGSGGGGSELVLTQSPSVSAALGSPAKITCTLSSAHKTDTIDWYQQLQGEAPRYLMQVQSDGSYTKRPGVPDRFSGSSSGADRYLIIPSVQADDEADYYCGADYIGGYVFGGGTQLTVTGESKYGPPCPPCPAPEFLGGPSVFLFPPKPKDTLMISRTPEVTCVVVDVSQEDPEVQFNWYVDGVEVHNAKTKPREEQFNSTYRVVSVLTVLHQDWLNGKEYKCKVSNKGLPSSIEKTISKAKGQPREPQVYTLPPSQEEMTKNQVSLTCLVKGFYPSDIAVEWESNGQPENNYKTTPPVLDSDGSFFLYSRLTVDKSRWQEGNVFSCSVMHEALHNHYTQKSLSLSLGKMFWVLVVVGGVLACYSLLVTVAFIIFWVKRGRKKLLYIFKQPFMRPVQTTQEEDGCSCRFPEEEEGGCELRVKFSRSADAPAYQQGQNQLYNELNLGRREEYDVLDKRRGRDPEMGGKPRRKNPQEGLYNELQKDKMAEAYSEIGMKGERRRGKGHDGLYQGLSTATKDTYDALHMQALPPRLEGGGEGRGSLLTCGDVEENPGPRMLLLVTSLLLCELPHPAFLLIPRKVCNGIGIGEFKDSLSINATNIKHFKNCTSISGDLHILPVAFRGDSFTHTPPLDPQELDILKTVKEITGFLLIQAWPENRTDLHAFENLEIIRGRTKQHGQFSLAVVSLNITSLGLRSLKEISDGDVIISGNKNLCYANTINWKKLFGTSGQKTKIISNRGENSCKATGQVCHALCSPEGCWGPEPRDCVSCRNVSRGRECVDKCNLLEGEPREFVENSECIQCHPECLPQAMNITCTGRGPDNCIQCAHYIDGPHCVKTCPAGVMGENNTLVWKYADAGHVCHLCHPNCTYGCTGPGLEGCPTNGPKIPSIATGMVGALLLLLVVALGIGLFM

SEQ ID NO: 39 - DNA, 9721 bp, Artificial Sequence
  Synthetic
gttagaccagatctgagcctgggagctctctggctaactagggaacccactgcttaagcctcaataaagcttgccttgagtgcttcaagtagtgtgtgcccgtctgttgtgtgactctggtaactagagatccctcagacccttttagtcagtgtggaaaatctctagcagtggcgcccgaacagggacttgaaagcgaaagggaaaccagaggagctctctcgacgcaggactcggcttgctgaagcgcgcacggcaagaggcgaggggcggcgactggtgagtacgccaaaaattttgactagcggaggctagaaggagagagatgggtgcgagagcgtcagtattaagcgggggagaattagatcgatgggaaaaaattcggttaaggccagggggaaagaaaaaatataaattaaaacatatagtatgggcaagcagggagctagaacgattcgcagttaatcctggcctgttagaaacatcagaaggctgtagacaaatactgggacagctacaaccatcccttcagacaggatcagaagaacttagatcattatataatacagtagcaaccctctattgtgtgcatcaaaggatagagataaaagacaccaaggaagctttagacaagatagaggaagagcaaaacaaaagtaagaaaaaagcacagcaagcagcagctgacacaggacacagcaatcaggtcagccaaaattaccctatagtgcagaacatccaggggcaaatggtacatcaggccatatcacctagaactttaaatgcatgggtaaaagtagtagaagagaaggctttcagcccagaagtgatacccatgttttcagcattatcagaaggagccaccccacaagatttaaacaccatgctaaacacagtggggggacatcaagcagccatgcaaatgttaaaagagaccatcaatgaggaagctgcaggcaaagagaagagtggtgcagagagaaaaaagagcagtgggaataggagctttgttccttgggttcttgggagcagcaggaagcactatgggcgcagcgtcaatgacgctgacggtacaggccagacaattattgtctggtatagtgcagcagcagaacaatttgctgagggctattgaggcgcaacagcatctgttgcaactcacagtctggggcatcaagcagctccaggcaagaatcctggctgtggaaagatacctaaaggatcaacagctcctggggatttggggttgctctggaaaactcatttgcaccactgctgtgccttggatctacaaatggcagtattcatccacaattttaaaagaaaaggggggattggggggtacagtgcaggggaaagaatagtagacataatagcaacagacatacaaactaaagaattacaaaaacaaattacaaaaattcaaaattttcgggtttattacagggacagcagagatccagtttggggatcaattgcatgaagaatctgcttagggttaggcgttttgcgctgcttcgcgaggatctgcgatcgctccggtgcccgtcagtgggcagagcgcacatcgcccacagtccccgagaagttggggggaggggtcggcaattgaaccggtgcctagagaaggtggcgcggggtaaactgggaaagtgatgtcgtgtactggctccgcctttttcccgagggtgggggagaaccgtatataagtgcagtagtcgccgtgaacgttctttttcgcaacgggtttgccgccagaacacagctgaagcttcgaggggctcgcatctctccttcacgcgcccgccgccctacctgaggccgccatccacgccggttgagtcgcgttctgccgcctcccgcctgtggtgcctcctgaactgcgtccgccgtctaggtaagtttaaagctcaggtcgagaccgggcctttgtccggcgctcccttggagcctacctagactcagccggctctccacgctttgcctgaccctgcttgctcaactctacgtctttgtttcgttttctgttctgcgccgttacagatccaagctgtgaccggcgcctacggctagcgaattcctcgaggccaccatgctgctgctggtgacaagcctgctgctgtgcgagctgccccaccccgcctttctgctgatcccccaggaacagctcgtcgaaagcggcggcagactggtgacacctggcggcagcctgaccctgagctgcaaggccagcggcttcgacttcagcgcctactacatgagctgggtccgccaggcccctggcaagggactggaatggatcgccaccatctaccccagcagcggcaagacctactacgccacctgggtgaacggacggttcaccatctccagcgacaacgcccagaacaccgtggacctgcagatgaacagcctgacagccgccgaccgggccacctacttttgcgccagagacagctacgccgacgacggcgccctgttcaacatctggggccctggcaccctggtgacaatctctagcggcggaggcggatctggtggcggaggaagtggcggcggaggatctgagctggtgctgacccagagcccctctgtgtctgctgccctgggaagccctgccaagatcacctgtaccctgagcagcgcccacaagaccgacaccatcgactggtatcagcagctgcagggcgaggcccccagatacctgatgcaggtgcagagcgacggcagctacaccaagaggccaggcgtgcccgaccggttcagcggatctagctctggcgccgaccgctacctgatcatccccagcgtgcaggccgatgacgaggccgattactactgtggcgccgactacatcggcggctacgtgttcggcggaggcacccagctgaccgtgaccggcgagtctaagtacggaccgccctgccccccttgccctggccagcctcgcgagccccaggtgtacaccctgcctccctcccaggaagagatgaccaagaaccaggtgtccctgacctgcctggtgaagggcttctaccccagcgacatcgccgtggagtgggagagcaacggccagcctgagaacaactacaagaccacccctcccgtgctggacagcgacggcagcttcttcctgtacagccggctgaccgtggacaagagccggtggcaggaaggcaacgtctttagctgcagcgtgatgcacgaggccctgcacaaccactacacccagaagagcctgagcctgtccctgggcaagatgttctgggtgctggtggtggtgggcggggtgctggcctgctacagcctgctggtgacagtggccttcatcatcttttgggtgaaacggggcagaaagaaactcctgtatatattcaaacaaccatttatgagaccagtacaaactactcaagaggaagatggctgtagctgccgatttccagaagaagaagaaggaggatgtgaactgcgggtgaagttcagcagaagcgccgacgcccctgcctaccagcagggccagaatcagctgtacaacgagctgaacctgggcagaagggaagagtacgacgtcctggataagcggagaggccgggaccctgagatgggcggcaagcctcggcggaagaacccccaggaaggcctgtataacgaactgcagaaagacaagatggccgaggcctacagcgagatcggcatgaagggcgagcggaggcggggcaagggccacgacggcctgtatcagggcctgtccaccgccaccaaggatacctacgacgccctgcacatgcaggccctgcccccaaggctcgagggcggcggagagggcagaggaagtcttctaacatgcggtgacgtggaggagaatcccggccctaggatgcttctcctggtgacaagccttctgctctgtgagttaccacacccagcattcctcctgatcccacgcaaagtgtgtaacggaataggtattggtgaatttaaagactcactctccataaatgctacgaatattaaacacttcaaaaactgcacctccatcagtggcgatctccacatcctgccggtggcatttaggggtgactccttcacacatactcctcctctggatccacaggaactggatattctgaaaaccgtaaaggaaatcacagggtttttgctgattcaggcttggcctgaaaacaggacggacctccatgcctttgagaacctagaaatcatacgcggcaggaccaagcaacatggtcagttttctcttgcagtcgtcagcctgaacataacatccttgggattacgctccctcaaggagataagtgatggagatgtgataatttcaggaaacaaaaatttgtgctatgcaaatacaataaactggaaaaaactgtttgggacctccggtcagaaaaccaaaattataagcaacagaggtgaaaacagctgcaaggccacaggccaggtctgccatgccttgtgctcccccgagggctgctggggcccggagcccagggactgcgtctcttgccggaatgtcagccgaggcagggaatgcgtggacaagtgcaaccttctggagggtgagccaagggagtttgtggagaactctgagtgcatacagtgccacccagagtgcctgcctcaggccatgaacatcacctgcacaggacggggaccagacaactgtatccagtgtgcccactacattgacggcccccactgcgtcaagacctgcccggcaggagtcatgggagaaaacaacaccctggtctggaagtacgcagacgccggccatgtgtgccacctgtgccatccaaactgcacctacggatgcactgggccaggtcttgaaggctgtccaacgaatgggcctaagatcccgtccatcgccactgggatggtgggggccctcctcttgctgctggtggtggccctggggatcggcctcttcatgtgagcggccgctctagacccgggctgcaggaattcgatatcaagcttatcgataatcaacctctggattacaaaatttgtgaaagattgactggtattcttaactatgttgctccttttacgctatgtggatacgctgctttaatgcctttgtatcatgctattgcttcccgtatggctttcattttctcctccttgtataaatcctggttgctgtctctttatgaggagttgtggcccgttgtcaggcaacgtggcgtggtgtgcactgtgtttgctgacgcaacccccactggttggggcattgccaccacctgtcagctcctttccgggactttcgctttccccctccctattgccacggcggaactcatcgccgcctgccttgcccgctgctggacaggggctcggctgttgggcactgacaattccgtggtgttgtcggggaaatcatcgtcctttccttggctgctcgcctgtgttgccacctggattctgcgcgggacgtccttctgctacgtcccttcggccctcaatccagcggaccttccttcccgcggcctgctgccggctctgcggcctcttccgcgtcttcgccttcgccctcagacgagtcggatctccctttgggccgcctccccgcatcgataccgtcgactagccgtacctttaagaccaatgacttacaaggcagctgtagatcttagccactttttaaaagaaaaggggggactggaagggctaattcactcccaaagaagacaagatctgctttttgcctgtactgggtctctctggttagaccagatctgagcctgggagctctctggctaactagggaacccactgcttaagcctcaataaagcttgccttgagtgcttcaagtagtgtgtgcccgtctgttgtgtgactctggtaactagagatccctcagacccttttagtcagtgtggaaaatctctagcagaattcgatatcaagcttatcgataccgtcgacctcgagggggggcccggtacccaattcgccctatagtgagtcgtattacaattcactggccgtcgttttacaacgtcgtgactgggaaaaccctggcgttacccaacttaatcgccttgcagcacatccccctttcgccagctggcgtaatagcgaagaggcccgcaccgatcgcccttcccaacagttgcgcagcctgaatggcgaatggaaattgtaagcgttaatattttgttaaaattcgcgttaaatttttgttaaatcagctcattttttaaccaataggccgaaatcggcaaaatcccttataaatcaaaagaatagaccgagatagggttgagtgttgttccagtttggaacaagagtccactattaaagaacgtggactccaacgtcaaagggcgaaaaaccgtctatcagggcgatggcccactacgtgaaccatcaccctaatcaagttttttggggtcgaggtgccgtaaagcactaaatcggaaccctaaagggagcccccgatttagagcttgacggggaaagccggcgaacgtggcgagaaaggaagggaagaaagcgaaaggagcgggcgctagggcgctggcaagtgtagcggtcacgctgcgcgtaaccaccacacccgccgcgcttaatgcgccgctacagggcgcgtcaggtggcacttttcggggaaatgtgcgcggaacccctatttgtttatttttctaaatacattcaaatatgtatccgctcatgagacaataaccctgataaatgcttcaataatattgaaaaaggaagagtatgagtattcaacatttccgtgtcgcccttattcccttttttgcggcattttgccttcctgtttttgctcacccagaaacgctggtgaaagtaaaagatgctgaagatcagttgggtgcacgagtgggttacatcgaactggatctcaacagcggtaagatccttgagagttttcgccccgaagaacgttttccaatgatgagcacttttaaagttctgctatgtggcgcggtattatcccgtattgacgccgggcaagagcaactcggtcgccgcatacactattctcagaatgacttggttgagtactcaccagtcacagaaaagcatcttacggatggcatgacagtaagagaattatgcagtgctgccataaccatgagtgataacactgcggccaacttacttctgacaacgatcggaggaccgaaggagctaaccgcttttttgcacaacatgggggatcatgtaactcgccttgatcgttgggaaccggagctgaatgaagccataccaaacgacgagcgtgacaccacgatgcctgtagcaatggcaacaacgttgcgcaaactattaactggcgaactacttactctagcttcccggcaacaattaatagactggatggaggcggataaagttgcaggaccacttctgcgctcggcccttccggctggctggtttattgctgataaatctggagccggtgagcgtgggtctcgcggtatcattgcagcactggggccagatggtaagccctcccgtatcgtagttatctacacgacggggagtcaggcaactatggatgaacgaaatagacagatcgctgagataggtgcctcactgattaagcattggtaactgtcagaccaagtttactcatatatactttagattgatttaaaacttcatttttaatttaaaaggatctaggtgaagatcctttttgataatctcatgaccaaaatcccttaacgtgagttttcgttccactgagcgtcagaccccgtagaaaagatcaaaggatcttcttgagatcctttttttctgcgcgtaatctgctgcttgcaaacaaaaaaaccaccgctaccagcggtggtttgtttgccggatcaagagctaccaactctttttccgaaggtaactggcttcagcagagcgcagataccaaatactgttcttctagtgtagccgtagttaggccaccacttcaagaactctgtagcaccgcctacatacctcgctctgctaatcctgttaccagtggctgctgccagtggcgataagtcgtgtcttaccgggttggactcaagacgatagttaccggataaggcgcagcggtcgggctgaacggggggttcgtgcacacagcccagcttggagcgaacgacctacaccgaactgagatacctacagcgtgagctatgagaaagcgccacgcttcccgaagggagaaaggcggacaggtatccggtaagcggcagggtcggaacaggagagcgcacgagggagcttccagggggaaacgcctggtatctttatagtcctgtcgggtttcgccacctctgacttgagcgtcgatttttgtgatgctcgtcaggggggcggagcctatggaaaaacgccagcaacgcggcctttttacggttcctggccttttgctggccttttgctcacatgttctttcctgcgttatcccctgattctgtggataaccgtattaccgcctttgagtgagctgataccgctcgccgcagccgaacgaccgagcgcagcgagtcagtgagcgaggaagcggaagagcgcccaatacgcaaaccgcctctccccgcgcgttggccgattcattaatgcagctggcacgacaggtttcccgactggaaagcgggcagtgagcgcaacgcaattaatgtgagttagctcactcattaggcaccccaggctttacactttatgcttccggctcgtatgttgtgtggaattgtgagcggataacaatttcacacaggaaacagctatgaccatgattacgccaagctcgaaattaaccctcactaaagggaacaaaagctggagctccaccgcggtggcggcctcgaggtcgagatccggtcgaccagcaaccatagtcccgcccctaactccgcccatcccgcccctaactccgcccagttccgcccattctccgccccatggctgactaattttttttatttatgcagaggccgaggccgcctcggcctctgagctattccagaagtagtgaggaggcttttttggaggcctaggcttttgcaaaaagcttcgacggtatcgattggctcatgtccaacattaccgccatgttgacattgattattgactagttattaatagtaatcaattacggggtcattagttcatagcccatatatggagttccgcgttacataacttacggtaaatggcccgcctggctgaccgcccaacgacccccgcccattgacgtcaataatgacgtatgttcccatagtaacgccaatagggactttccattgacgtcaatgggtggagtatttacggtaaactgcccacttggcagtacatcaagtgtatcatatgccaagtacgccccctattgacgtcaatgacggtaaatggcccgcctggcattatgcccagtacatgaccttatgggactttcctacttggcagtacatctacgtattagtcatcgctattaccatggtgatgcggttttggcagtacatcaatgggcgtggatagcggtttgactcacggggatttccaagtctccaccccattgacgtcaatgggagtttgttttggcaccaaaatcaacgggactttccaaaatgtcgtaacaactccgccccattgacgcaaatgggcggtaggcgtgtacggaattcggagtggcgagccctcagatcctgcatataagcagctgctttttgcctgtactgggtctctctg

SEQ ID NO: 40 - protein, 952 aa, Artificial Sequence
  Synthetic
MLLLVTSLLLCELPHPAFLLIPQEQLVESGGRLVTPGGSLTLSCKASGFDFSAYYMSWVRQAPGKGLEWIATIYPSSGKTYYATWVNGRFTISSDNAQNTVDLQMNSLTAADRATYFCARDSYADDGALFNIWGPGTLVTISSGGGGSGGGGSGGGGSELVLTQSPSVSAALGSPAKITCTLSSAHKTDTIDWYQQLQGEAPRYLMQVQSDGSYTKRPGVPDRFSGSSSGADRYLIIPSVQADDEADYYCGADYIGGYVFGGGTQLTVTGESKYGPPCPPCPGQPREPQVYTLPPSQEEMTKNQVSLTCLVKGFYPSDIAVEWESNGQPENNYKTTPPVLDSDGSFFLYSRLTVDKSRWQEGNVFSCSVMHEALHNHYTQKSLSLSLGKMFWVLVVVGGVLACYSLLVTVAFIIFWVKRGRKKLLYIFKQPFMRPVQTTQEEDGCSCRFPEEEEGGCELRVKFSRSADAPAYQQGQNQLYNELNLGRREEYDVLDKRRGRDPEMGGKPRRKNPQEGLYNELQKDKMAEAYSEIGMKGERRRGKGHDGLYQGLSTATKDTYDALHMQALPPRLEGGGEGRGSLLTCGDVEENPGPRMLLLVTSLLLCELPHPAFLLIPRKVCNGIGIGEFKDSLSINATNIKHFKNCTSISGDLHILPVAFRGDSFTHTPPLDPQELDILKTVKEITGFLLIQAWPENRTDLHAFENLEIIRGRTKQHGQFSLAVVSLNITSLGLRSLKEISDGDVIISGNKNLCYANTINWKKLFGTSGQKTKIISNRGENSCKATGQVCHALCSPEGCWGPEPRDCVSCRNVSRGRECVDKCNLLEGEPREFVENSECIQCHPECLPQAMNITCTGRGPDNCIQCAHYIDGPHCVKTCPAGVMGENNTLVWKYADAGHVCHLCHPNCTYGCTGPGLEGCPTNGPKIPSIATGMVGALLLLLVVALGIGLFM

SEQ ID NO: 41 - DNA, 9400 bp, Artificial Sequence
  Synthetic
gttagaccagatctgagcctgggagctctctggctaactagggaacccactgcttaagcctcaataaagcttgccttgagtgcttcaagtagtgtgtgcccgtctgttgtgtgactctggtaactagagatccctcagacccttttagtcagtgtggaaaatctctagcagtggcgcccgaacagggacttgaaagcgaaagggaaaccagaggagctctctcgacgcaggactcggcttgctgaagcgcgcacggcaagaggcgaggggcggcgactggtgagtacgccaaaaattttgactagcggaggctagaaggagagagatgggtgcgagagcgtcagtattaagcgggggagaattagatcgatgggaaaaaattcggttaaggccagggggaaagaaaaaatataaattaaaacatatagtatgggcaagcagggagctagaacgattcgcagttaatcctggcctgttagaaacatcagaaggctgtagacaaatactgggacagctacaaccatcccttcagacaggatcagaagaacttagatcattatataatacagtagcaaccctctattgtgtgcatcaaaggatagagataaaagacaccaaggaagctttagacaagatagaggaagagcaaaacaaaagtaagaaaaaagcacagcaagcagcagctgacacaggacacagcaatcaggtcagccaaaattaccctatagtgcagaacatccaggggcaaatggtacatcaggccatatcacctagaactttaaatgcatgggtaaaagtagtagaagagaaggctttcagcccagaagtgatacccatgttttcagcattatcagaaggagccaccccacaagatttaaacaccatgctaaacacagtggggggacatcaagcagccatgcaaatgttaaaagagaccatcaatgaggaagctgcaggcaaagagaagagtggtgcagagagaaaaaagagcagtgggaataggagctttgttccttgggttcttgggagcagcaggaagcactatgggcgcagcgtcaatgacgctgacggtacaggccagacaattattgtctggtatagtgcagcagcagaacaatttgctgagggctattgaggcgcaacagcatctgttgcaactcacagtctggggcatcaagcagctccaggcaagaatcctggctgtggaaagatacctaaaggatcaacagctcctggggatttggggttgctctggaaaactcatttgcaccactgctgtgccttggatctacaaatggcagtattcatccacaattttaaaagaaaaggggggattggggggtacagtgcaggggaaagaatagtagacataatagcaacagacatacaaactaaagaattacaaaaacaaattacaaaaattcaaaattttcgggtttattacagggacagcagagatccagtttggggatcaattgcatgaagaatctgcttagggttaggcgttttgcgctgcttcgcgaggatctgcgatcgctccggtgcccgtcagtgggcagagcgcacatcgcccacagtccccgagaagttggggggaggggtcggcaattgaaccggtgcctagagaaggtggcgcggggtaaactgggaaagtgatgtcgtgtactggctccgcctttttcccgagggtgggggagaaccgtatataagtgcagtagtcgccgtgaacgttctttttcgcaacgggtttgccgccagaacacagctgaagcttcgaggggctcgcatctctccttcacgcgcccgccgccctacctgaggccgccatccacgccggttgagtcgcgttctgccgcctcccgcctgtggtgcctcctgaactgcgtccgccgtctaggtaagtttaaagctcaggtcgagaccgggcctttgtccggcgctcccttggagcctacctagactcagccggctctccacgctttgcctgaccctgcttgctcaactctacgtctttgtttcgttttctgttctgcgccgttacagatccaagctgtgaccggcgcctacggctagcgaattcctcgaggccaccatgctgctgctggtgacaagcctgctgctgtgcgagctgccccaccccgcctttctgctgatcccccaggaacagctcgtcgaaagcggcggcagactggtgacacctggcggcagcctgaccctgagctgcaaggccagcggcttcgacttcagcgcctactacatgagctgggtccgccaggcccctggcaagggactggaatggatcgccaccatctaccccagcagcggcaagacctactacgccacctgggtgaacggacggttcaccatctccagcgacaacgcccagaacaccgtggacctgcagatgaacagcctgacagccgccgaccgggccacctacttttgcgccagagacagctacgccgacgacggcgccctgttcaacatctggggccctggcaccctggtgacaatctctagcggcggaggcggatctggtggcggaggaagtggcggcggaggatctgagctggtgctgacccagagcccctctgtgtctgctgccctgggaagccctgccaagatcacctgtaccctgagcagcgcccacaagaccgacaccatcgactggtatcagcagctgcagggcgaggcccccagatacctgatgcaggtgcagagcgacggcagctacaccaagaggccaggcgtgcccgaccggttcagcggatctagctctggcgccgaccgctacctgatcatccccagcgtgcaggccgatgacgaggccgattactactgtggcgccgactacatcggcggctacgtgttcggcggaggcacccagctgaccgtgaccggcgagtctaagtacggaccgccctgccccccttgccctatgttctgggtgctggtggtggtgggcggggtgctggcctgctacagcctgctggtgacagtggccttcatcatcttttgggtgaaacggggcagaaagaaactcctgtatatattcaaacaaccatttatgagaccagtacaaactactcaagaggaagatggctgtagctgccgatttccagaagaagaagaaggaggatgtgaactgcgggtgaagttcagcagaagcgccgacgcccctgcctaccagcagggccagaatcagctgtacaacgagctgaacctgggcagaagggaagagtacgacgtcctggataagcggagaggccgggaccctgagatgggcggcaagcctcggcggaagaacccccaggaaggcctgtataacgaactgcagaaagacaagatggccgaggcctacagcgagatcggcatgaagggcgagcggaggcggggcaagggccacgacggcctgtatcagggcctgtccaccgccaccaaggatacctacgacgccctgcacatgcaggccctgcccccaaggctcgagggcggcggagagggcagaggaagtcttctaacatgcggtgacgtggaggagaatcccggccctaggatgcttctcctggtgacaagccttctgctctgtgagttaccacacccagcattcctcctgatcccacgcaaagtgtgtaacggaataggtattggtgaatttaaagactcactctccataaatgctacgaatattaaacacttcaaaaactgcacctccatcagtggcgatctccacatcctgccggtggcatttaggggtgactccttcacacatactcctcctctggatccacaggaactggatattctgaaaaccgtaaaggaaatcacagggtttttgctgattcaggcttggcctgaaaacaggacggacctccatgcctttgagaacctagaaatcatacgcggcaggaccaagcaacatggtcagttttctcttgcagtcgtcagcctgaacataacatccttgggattacgctccctcaaggagataagtgatggagatgtgataatttcaggaaacaaaaatttgtgctatgcaaatacaataaactggaaaaaactgtttgggacctccggtcagaaaaccaaaattataagcaacagaggtgaaaacagctgcaaggccacaggccaggtctgccatgccttgtgctcccccgagggctgctggggcccggagcccagggactgcgtctcttgccggaatgtcagccgaggcagggaatgcgtggacaagtgcaaccttctggagggtgagccaagggagtttgtggagaactctgagtgcatacagtgccacccagagtgcctgcctcaggccatgaacatcacctgcacaggacggggaccagacaactgtatccagtgtgcccactacattgacggcccccactgcgtcaagacctgcccggcaggagtcatgggagaaaacaacaccctggtctggaagtacgcagacgccggccatgtgtgccacctgtgccatccaaactgcacctacggatgcactgggccaggtcttgaaggctgtccaacgaatgggcctaagatcccgtccatcgccactgggatggtgggggccctcctcttgctgctggtggtggccctggggatcggcctcttcatgtgagcggccgctctagacccgggctgcaggaattcgatatcaagcttatcgataatcaacctctggattacaaaatttgtgaaagattgactggtattcttaactatgttgctccttttacgctatgtggatacgctgctttaatgcctttgtatcatgctattgcttcccgtatggctttcattttctcctccttgtataaatcctggttgctgtctctttatgaggagttgtggcccgttgtcaggcaacgtggcgtggtgtgcactgtgtttgctgacgcaacccccactggttggggcattgccaccacctgtcagctcctttccgggactttcgctttccccctccctattgccacggcggaactcatcgccgcctgccttgcccgctgctggacaggggctcggctgttgggcactgacaattccgtggtgttgtcggggaaatcatcgtcctttccttggctgctcgcctgtgttgccacctggattctgcgcgggacgtccttctgctacgtcccttcggccctcaatccagcggaccttccttcccgcggcctgctgccggctctgcggcctcttccgcgtcttcgccttcgccctcagacgagtcggatctccctttgggccgcctccccgcatcgataccgtcgactagccgtacctttaagaccaatgacttacaaggcagctgtagatcttagccactttttaaaagaaaaggggggactggaagggctaattcactcccaaagaagacaagatctgctttttgcctgtactgggtctctctggttagaccagatctgagcctgggagctctctggctaactagggaacccactgcttaagcctcaataaagcttgccttgagtgcttcaagtagtgtgtgcccgtctgttgtgtgactctggtaactagagatccctcagacccttttagtcagtgtggaaaatctctagcagaattcgatatcaagcttatcgataccgtcgacctcgagggggggcccggtacccaattcgccctatagtgagtcgtattacaattcactggccgtcgttttacaacgtcgtgactgggaaaaccctggcgttacccaacttaatcgccttgcagcacatccccctttcgccagctggcgtaatagcgaagaggcccgcaccgatcgcccttcccaacagttgcgcagcctgaatggcgaatggaaattgtaagcgttaatattttgttaaaattcgcgttaaatttttgttaaatcagctcattttttaaccaataggccgaaatcggcaaaatcccttataaatcaaaagaatagaccgagatagggttgagtgttgttccagtttggaacaagagtccactattaaagaacgtggactccaacgtcaaagggcgaaaaaccgtctatcagggcgatggcccactacgtgaaccatcaccctaatcaagttttttggggtcgaggtgccgtaaagcactaaatcggaaccctaaagggagcccccgatttagagcttgacggggaaagccggcgaacgtggcgagaaaggaagggaagaaagcgaaaggagcgggcgctagggcgctggcaagtgtagcggtcacgctgcgcgtaaccaccacacccgccgcgcttaatgcgccgctacagggcgcgtcaggtggcacttttcggggaaatgtgcgcggaacccctatttgtttatttttctaaatacattcaaatatgtatccgctcatgagacaataaccctgataaatgcttcaataatattgaaaaaggaagagtatgagtattcaacatttccgtgtcgcccttattcccttttttgcggcattttgccttcctgtttttgctcacccagaaacgctggtgaaagtaaaagatgctgaagatcagttgggtgcacgagtgggttacatcgaactggatctcaacagcggtaagatccttgagagttttcgccccgaagaacgttttccaatgatgagcacttttaaagttctgctatgtggcgcggtattatcccgtattgacgccgggcaagagcaactcggtcgccgcatacactattctcagaatgacttggttgagtactcaccagtcacagaaaagcatcttacggatggcatgacagtaagagaattatgcagtgctgccataaccatgagtgataacactgcggccaacttacttctgacaacgatcggaggaccgaaggagctaaccgcttttttgcacaacatgggggatcatgtaactcgccttgatcgttgggaaccggagctgaatgaagccataccaaacgacgagcgtgacaccacgatgcctgtagcaatggcaacaacgttgcgcaaactattaactggcgaactacttactctagcttcccggcaacaattaatagactggatggaggcggataaagttgcaggaccacttctgcgctcggcccttccggctggctggtttattgctgataaatctggagccggtgagcgtgggtctcgcggtatcattgcagcactggggccagatggtaagccctcccgtatcgtagttatctacacgacggggagtcaggcaactatggatgaacgaaatagacagatcgctgagataggtgcctcactgattaagcattggtaactgtcagaccaagtttactcatatatactttagattgatttaaaacttcatttttaatttaaaaggatctaggtgaagatcctttttgataatctcatgaccaaaatcccttaacgtgagttttcgttccactgagcgtcagaccccgtagaaaagatcaaaggatcttcttgagatcctttttttctgcgcgtaatctgctgcttgcaaacaaaaaaaccaccgctaccagcggtggtttgtttgccggatcaagagctaccaactctttttccgaaggtaactggcttcagcagagcgcagataccaaatactgttcttctagtgtagccgtagttaggccaccacttcaagaactctgtagcaccgcctacatacctcgctctgctaatcctgttaccagtggctgctgccagtggcgataagtcgtgtcttaccgggttggactcaagacgatagttaccggataaggcgcagcggtcgggctgaacggggggttcgtgcacacagcccagcttggagcgaacgacctacaccgaactgagatacctacagcgtgagctatgagaaagcgccacgcttcccgaagggagaaaggcggacaggtatccggtaagcggcagggtcggaacaggagagcgcacgagggagcttccagggggaaacgcctggtatctttatagtcctgtcgggtttcgccacctctgacttgagcgtcgatttttgtgatgctcgtcaggggggcggagcctatggaaaaacgccagcaacgcggcctttttacggttcctggccttttgctggccttttgctcacatgttctttcctgcgttatcccctgattctgtggataaccgtattaccgcctttgagtgagctgataccgctcgccgcagccgaacgaccgagcgcagcgagtcagtgagcgaggaagcggaagagcgcccaatacgcaaaccgcctctccccgcgcgttggccgattcattaatgcagctggcacgacaggtttcccgactggaaagcgggcagtgagcgcaacgcaattaatgtgagttagctcactcattaggcaccccaggctttacactttatgcttccggctcgtatgttgtgtggaattgtgagcggataacaatttcacacaggaaacagctatgaccatgattacgccaagctcgaaattaaccctcactaaagggaacaaaagctggagctccaccgcggtggcggcctcgaggtcgagatccggtcgaccagcaaccatagtcccgcccctaactccgcccatcccgcccctaactccgcccagttccgcccattctccgccccatggctgactaattttttttatttatgcagaggccgaggccgcctcggcctctgagctattccagaagtagtgaggaggcttttttggaggcctaggcttttgcaaaaagcttcgacggtatcgattggctcatgtccaacattaccgccatgttgacattgattattgactagttattaatagtaatcaattacggggtcattagttcatagcccatatatggagttccgcgttacataacttacggtaaatggcccgcctggctgaccgcccaacgacccccgcccattgacgtcaataatgacgtatgttcccatagtaacgccaatagggactttccattgacgtcaatgggtggagtatttacggtaaactgcccacttggcagtacatcaagtgtatcatatgccaagtacgccccctattgacgtcaatgacggtaaatggcccgcctggcattatgcccagtacatgaccttatgggactttcctacttggcagtacatctacgtattagtcatcgctattaccatggtgatgcggttttggcagtacatcaatgggcgtggatagcggtttgactcacggggatttccaagtctccaccccattgacgtcaatgggagtttgttttggcaccaaaatcaacgggactttccaaaatgtcgtaacaactccgccccattgacgcaaatgggcggtaggcgtgtacggaattcggagtggcgagccctcagatcctgcatataagcagctgctttttgcctgtactgggtctctctg

SEQ ID NO: 42 - protein, 845 aa, Artificial Sequence
  Synthetic
MLLLVTSLLLCELPHPAFLLIPQEQLVESGGRLVTPGGSLTLSCKASGFDFSAYYMSWVRQAPGKGLEWIATIYPSSGKTYYATWVNGRFTISSDNAQNTVDLQMNSLTAADRATYFCARDSYADDGALFNIWGPGTLVTISSGGGGSGGGGSGGGGSELVLTQSPSVSAALGSPAKITCTLSSAHKTDTIDWYQQLQGEAPRYLMQVQSDGSYTKRPGVPDRFSGSSSGADRYLIIPSVQADDEADYYCGADYIGGYVFGGGTQLTVTGESKYGPPCPPCPMFWVLVVVGGVLACYSLLVTVAFIIFWVKRGRKKLLYIFKQPFMRPVQTTQEEDGCSCRFPEEEEGGCELRVKFSRSADAPAYQQGQNQLYNELNLGRREEYDVLDKRRGRDPEMGGKPRRKNPQEGLYNELQKDKMAEAYSEIGMKGERRRGKGHDGLYQGLSTATKDTYDALHMQALPPRLEGGGEGRGSLLTCGDVEENPGPRMLLLVTSLLLCELPHPAFLLIPRKVCNGIGIGEFKDSLSINATNIKHFKNCTSISGDLHILPVAFRGDSFTHTPPLDPQELDILKTVKEITGFLLIQAWPENRTDLHAFENLEIIRGRTKQHGQFSLAVVSLNITSLGLRSLKEISDGDVIISGNKNLCYANTINWKKLFGTSGQKTKIISNRGENSCKATGQVCHALCSPEGCWGPEPRDCVSCRNVSRGRECVDKCNLLEGEPREFVENSECIQCHPECLPQAMNITCTGRGPDNCIQCAHYIDGPHCVKTCPAGVMGENNTLVWKYADAGHVCHLCHPNCTYGCTGPGLEGCPTNGPKIPSIATGMVGALLLLLVVALGIGLFM

SEQ ID NO: 43 - DNA, 10015 bp, Artificial Sequence
  Synthetic
gttagaccagatctgagcctgggagctctctggctaactagggaacccactgcttaagcctcaataaagcttgccttgagtgcttcaagtagtgtgtgcccgtctgttgtgtgactctggtaactagagatccctcagacccttttagtcagtgtggaaaatctctagcagtggcgcccgaacagggacttgaaagcgaaagggaaaccagaggagctctctcgacgcaggactcggcttgctgaagcgcgcacggcaagaggcgaggggcggcgactggtgagtacgccaaaaattttgactagcggaggctagaaggagagagatgggtgcgagagcgtcagtattaagcgggggagaattagatcgatgggaaaaaattcggttaaggccagggggaaagaaaaaatataaattaaaacatatagtatgggcaagcagggagctagaacgattcgcagttaatcctggcctgttagaaacatcagaaggctgtagacaaatactgggacagctacaaccatcccttcagacaggatcagaagaacttagatcattatataatacagtagcaaccctctattgtgtgcatcaaaggatagagataaaagacaccaaggaagctttagacaagatagaggaagagcaaaacaaaagtaagaaaaaagcacagcaagcagcagctgacacaggacacagcaatcaggtcagccaaaattaccctatagtgcagaacatccaggggcaaatggtacatcaggccatatcacctagaactttaaatgcatgggtaaaagtagtagaagagaaggctttcagcccagaagtgatacccatgttttcagcattatcagaaggagccaccccacaagatttaaacaccatgctaaacacagtggggggacatcaagcagccatgcaaatgttaaaagagaccatcaatgaggaagctgcaggcaaagagaagagtggtgcagagagaaaaaagagcagtgggaataggagctttgttccttgggttcttgggagcagcaggaagcactatgggcgcagcgtcaatgacgctgacggtacaggccagacaattattgtctggtatagtgcagcagcagaacaatttgctgagggctattgaggcgcaacagcatctgttgcaactcacagtctggggcatcaagcagctccaggcaagaatcctggctgtggaaagatacctaaaggatcaacagctcctggggatttggggttgctctggaaaactcatttgcaccactgctgtgccttggatctacaaatggcagtattcatccacaattttaaaagaaaaggggggattggggggtacagtgcaggggaaagaatagtagacataatagcaacagacatacaaactaaagaattacaaaaacaaattacaaaaattcaaaattttcgggtttattacagggacagcagagatccagtttggggatcaattgcatgaagaatctgcttagggttaggcgttttgcgctgcttcgcgaggatctgcgatcgctccggtgcccgtcagtgggcagagcgcacatcgcccacagtccccgagaagttggggggaggggtcggcaattgaaccggtgcctagagaaggtggcgcggggtaaactgggaaagtgatgtcgtgtactggctccgcctttttcccgagggtgggggagaaccgtatataagtgcagtagtcgccgtgaacgttctttttcgcaacgggtttgccgccagaacacagctgaagcttcgaggggctcgcatctctccttcacgcgcccgccgccctacctgaggccgccatccacgccggttgagtcgcgttctgccgcctcccgcctgtggtgcctcctgaactgcgtccgccgtctaggtaagtttaaagctcaggtcgagaccgggcctttgtccggcgctcccttggagcctacctagactcagccggctctccacgctttgcctgaccctgcttgctcaactctacgtctttgtttcgttttctgttctgcgccgttacagatccaagctgtgaccggcgcctacggctagcgaattcgccaccatgctgctgctggtgacaagcctgctgctgtgcgagctgccccaccccgcctttctgctgatcccccagagcgtgaaagagtccgagggcgacctggtcacaccagccggcaacctgaccctgacctgtaccgccagcggcagcgacatcaacgactaccccatctcttgggtccgccaggctcctggcaagggactggaatggatcggcttcatcaacagcggcggcagcacttggtacgccagctgggtcaaaggccggttcaccatcagccggaccagcaccaccgtggacctgaagatgacaagcctgaccaccgacgacaccgccacctacttttgcgccagaggctacagcacctactacggcgacttcaacatctggggccctggcaccctggtcacaatctctagcggcggaggcggcagcggaggtggaggaagtggcggcggaggatccgagctggtcatgacccagacccccagcagcacatctggcgccgtgggcggcaccgtgaccatcaattgccaggccagccagagcatcgacagcaacctggcctggttccagcagaagcccggccagccccccaccctgctgatctacagagcctccaacctggccagcggcgtgccaagcagattcagcggcagcagatctggcaccgagtacaccctgaccatctccggcgtgcagagagaggacgccgctacctattactgcctgggcggcgtgggcaacgtgtcctacagaaccagcttcggcggaggtactgaggtggtcgtcaaatacggaccgccctgccccccttgccctgcccccgagttcctgggcggacccagcgtgttcctgttcccccccaagcccaaggacaccctgatgatcagccggacccccgaggtgacctgcgtggtggtggacgtgagccaggaagatcccgaggtccagttcaattggtacgtggacggcgtggaagtgcacaacgccaagaccaagcccagagaggaacagttcaacagcacctaccgggtggtgtctgtgctgaccgtgctgcaccaggactggctgaacggcaaagaatacaagtgcaaggtgtccaacaagggcctgcccagcagcatcgaaaagaccatcagcaaggccaagggccagcctcgcgagccccaggtgtacaccctgcctccctcccaggaagagatgaccaagaaccaggtgtccctgacctgcctggtgaagggcttctaccccagcgacatcgccgtggagtgggagagcaacggccagcctgagaacaactacaagaccacccctcccgtgctggacagcgacggcagcttcttcctgtacagccggctgaccgtggacaagagccggtggcaggaaggcaacgtctttagctgcagcgtgatgcacgaggccctgcacaaccactacacccagaagagcctgagcctgtccctgggcaagatgttctgggtgctggtggtggtgggcggggtgctggcctgctacagcctgctggtgacagtggccttcatcatcttttgggtgaaacggggcagaaagaaactcctgtatatattcaaacaaccatttatgagaccagtacaaactactcaagaggaagatggctgtagctgccgatttccagaagaagaagaaggaggatgtgaactgcgggtgaagttcagcagaagcgccgacgcccctgcctaccagcagggccagaatcagctgtacaacgagctgaacctgggcagaagggaagagtacgacgtcctggataagcggagaggccgggaccctgagatgggcggcaagcctcggcggaagaacccccaggaaggcctgtataacgaactgcagaaagacaagatggccgaggcctacagcgagatcggcatgaagggcgagcggaggcggggcaagggccacgacggcctgtatcagggcctgtccaccgccaccaaggatacctacgacgccctgcacatgcaggccctgcccccaaggctcgagggcggcggagagggcagaggaagtcttctaacatgcggtgacgtggaggagaatcccggccctaggatgcttctcctggtgacaagccttctgctctgtgagttaccacacccagcattcctcctgatcccacgcaaagtgtgtaacggaataggtattggtgaatttaaagactcactctccataaatgctacgaatattaaacacttcaaaaactgcacctccatcagtggcgatctccacatcctgccggtggcatttaggggtgactccttcacacatactcctcctctggatccacaggaactggatattctgaaaaccgtaaaggaaatcacagggtttttgctgattcaggcttggcctgaaaacaggacggacctccatgcctttgagaacctagaaatcatacgcggcaggaccaagcaacatggtcagttttctcttgcagtcgtcagcctgaacataacatccttgggattacgctccctcaaggagataagtgatggagatgtgataatttcaggaaacaaaaatttgtgctatgcaaatacaataaactggaaaaaactgtttgggacctccggtcagaaaaccaaaattataagcaacagaggtgaaaacagctgcaaggccacaggccaggtctgccatgccttgtgctcccccgagggctgctggggcccggagcccagggactgcgtctcttgccggaatgtcagccgaggcagggaatgcgtggacaagtgcaaccttctggagggtgagccaagggagtttgtggagaactctgagtgcatacagtgccacccagagtgcctgcctcaggccatgaacatcacctgcacaggacggggaccagacaactgtatccagtgtgcccactacattgacggcccccactgcgtcaagacctgcccggcaggagtcatgggagaaaacaacaccctggtctggaagtacgcagacgccggccatgtgtgccacctgtgccatccaaactgcacctacggatgcactgggccaggtcttgaaggctgtccaacgaatgggcctaagatcccgtccatcgccactgggatggtgggggccctcctcttgctgctggtggtggccctggggatcggcctcttcatgtgagcggccgctctagacccgggctgcaggaattcgatatcaagcttatcgataatcaacctctggattacaaaatttgtgaaagattgactggtattcttaactatgttgctccttttacgctatgtggatacgctgctttaatgcctttgtatcatgctattgcttcccgtatggctttcattttctcctccttgtataaatcctggttgctgtctctttatgaggagttgtggcccgttgtcaggcaacgtggcgtggtgtgcactgtgtttgctgacgcaacccccactggttggggcattgccaccacctgtcagctcctttccgggactttcgctttccccctccctattgccacggcggaactcatcgccgcctgccttgcccgctgctggacaggggctcggctgttgggcactgacaattccgtggtgttgtcggggaaatcatcgtcctttccttggctgctcgcctgtgttgccacctggattctgcgcgggacgtccttctgctacgtcccttcggccctcaatccagcggaccttccttcccgcggcctgctgccggctctgcggcctcttccgcgtcttcgccttcgccctcagacgagtcggatctccctttgggccgcctccccgcatcgataccgtcgactagccgtacctttaagaccaatgacttacaaggcagctgtagatcttagccactttttaaaagaaaaggggggactggaagggctaattcactcccaaagaagacaagatctgctttttgcctgtactgggtctctctggttagaccagatctgagcctgggagctctctggctaactagggaacccactgcttaagcctcaataaagcttgccttgagtgcttcaagtagtgtgtgcccgtctgttgtgtgactctggtaactagagatccctcagacccttttagtcagtgtggaaaatctctagcagaattcgatatcaagcttatcgataccgtcgacctcgagggggggcccggtacccaattcgccctatagtgagtcgtattacaattcactggccgtcgttttacaacgtcgtgactgggaaaaccctggcgttacccaacttaatcgccttgcagcacatccccctttcgccagctggcgtaatagcgaagaggcccgcaccgatcgcccttcccaacagttgcgcagcctgaatggcgaatggaaattgtaagcgttaatattttgttaaaattcgcgttaaatttttgttaaatcagctcattttttaaccaataggccgaaatcggcaaaatcccttataaatcaaaagaatagaccgagatagggttgagtgttgttccagtttggaacaagagtccactattaaagaacgtggactccaacgtcaaagggcgaaaaaccgtctatcagggcgatggcccactacgtgaaccatcaccctaatcaagttttttggggtcgaggtgccgtaaagcactaaatcggaaccctaaagggagcccccgatttagagcttgacggggaaagccggcgaacgtggcgagaaaggaagggaagaaagcgaaaggagcgggcgctagggcgctggcaagtgtagcggtcacgctgcgcgtaaccaccacacccgccgcgcttaatgcgccgctacagggcgcgtcaggtggcacttttcggggaaatgtgcgcggaacccctatttgtttatttttctaaatacattcaaatatgtatccgctcatgagacaataaccctgataaatgcttcaataatattgaaaaaggaagagtatgagtattcaacatttccgtgtcgcccttattcccttttttgcggcattttgccttcctgtttttgctcacccagaaacgctggtgaaagtaaaagatgctgaagatcagttgggtgcacgagtgggttacatcgaactggatctcaacagcggtaagatccttgagagttttcgccccgaagaacgttttccaatgatgagcacttttaaagttctgctatgtggcgcggtattatcccgtattgacgccgggcaagagcaactcggtcgccgcatacactattctcagaatgacttggttgagtactcaccagtcacagaaaagcatcttacggatggcatgacagtaagagaattatgcagtgctgccataaccatgagtgataacactgcggccaacttacttctgacaacgatcggaggaccgaaggagctaaccgcttttttgcacaacatgggggatcatgtaactcgccttgatcgttgggaaccggagctgaatgaagccataccaaacgacgagcgtgacaccacgatgcctgtagcaatggcaacaacgttgcgcaaactattaactggcgaactacttactctagcttcccggcaacaattaatagactggatggaggcggataaagttgcaggaccacttctgcgctcggcccttccggctggctggtttattgctgataaatctggagccggtgagcgtgggtctcgcggtatcattgcagcactggggccagatggtaagccctcccgtatcgtagttatctacacgacggggagtcaggcaactatggatgaacgaaatagacagatcgctgagataggtgcctcactgattaagcattggtaactgtcagaccaagtttactcatatatactttagattgatttaaaacttcatttttaatttaaaaggatctaggtgaagatcctttttgataatctcatgaccaaaatcccttaacgtgagttttcgttccactgagcgtcagaccccgtagaaaagatcaaaggatcttcttgagatcctttttttctgcgcgtaatctgctgcttgcaaacaaaaaaaccaccgctaccagcggtggtttgtttgccggatcaagagctaccaactctttttccgaaggtaactggcttcagcagagcgcagataccaaatactgttcttctagtgtagccgtagttaggccaccacttcaagaactctgtagcaccgcctacatacctcgctctgctaatcctgttaccagtggctgctgccagtggcgataagtcgtgtcttaccgggttggactcaagacgatagttaccggataaggcgcagcggtcgggctgaacggggggttcgtgcacacagcccagcttggagcgaacgacctacaccgaactgagatacctacagcgtgagctatgagaaagcgccacgcttcccgaagggagaaaggcggacaggtatccggtaagcggcagggtcggaacaggagagcgcacgagggagcttccagggggaaacgcctggtatctttatagtcctgtcgggtttcgccacctctgacttgagcgtcgatttttgtgatgctcgtcaggggggcggagcctatggaaaaacgccagcaacgcggcctttttacggttcctggccttttgctggccttttgctcacatgttctttcctgcgttatcccctgattctgtggataaccgtattaccgcctttgagtgagctgataccgctcgccgcagccgaacgaccgagcgcagcgagtcagtgagcgaggaagcggaagagcgcccaatacgcaaaccgcctctccccgcgcgttggccgattcattaatgcagctggcacgacaggtttcccgactggaaagcgggcagtgagcgcaacgcaattaatgtgagttagctcactcattaggcaccccaggctttacactttatgcttccggctcgtatgttgtgtggaattgtgagcggataacaatttcacacaggaaacagctatgaccatgattacgccaagctcgaaattaaccctcactaaagggaacaaaagctggagctccaccgcggtggcggcctcgaggtcgagatccggtcgaccagcaaccatagtcccgcccctaactccgcccatcccgcccctaactccgcccagttccgcccattctccgccccatggctgactaattttttttatttatgcagaggccgaggccgcctcggcctctgagctattccagaagtagtgaggaggcttttttggaggcctaggcttttgcaaaaagcttcgacggtatcgattggctcatgtccaacattaccgccatgttgacattgattattgactagttattaatagtaatcaattacggggtcattagttcatagcccatatatggagttccgcgttacataacttacggtaaatggcccgcctggctgaccgcccaacgacccccgcccattgacgtcaataatgacgtatgttcccatagtaacgccaatagggactttccattgacgtcaatgggtggagtatttacggtaaactgcccacttggcagtacatcaagtgtatcatatgccaagtacgccccctattgacgtcaatgacggtaaatggcccgcctggcattatgcccagtacatgaccttatgggactttcctacttggcagtacatctacgtattagtcatcgctattaccatggtgatgcggttttggcagtacatcaatgggcgtggatagcggtttgactcacggggatttccaagtctccaccccattgacgtcaatgggagtttgttttggcaccaaaatcaacgggactttccaaaatgtcgtaacaactccgccccattgacgcaaatgggcggtaggcgtgtacggaattcggagtggcgagccctcagatcctgcatataagcagctgctttttgcctgtactgggtctctctg

SEQ ID NO: 44 - protein, 1055 aa, Artificial Sequence [sequence omitted]

SEQ ID NO: 45 - DNA, 10015 bp, Artificial Sequence; identical to SEQ ID NO: 43
  Synthetic

SEQ ID NO: 46 - protein, 945 aa, Artificial Sequence
  Synthetic
MLLLVTSLLLCELPHPAFLLIPQSVKESEGDLVTPAGNLTLTCTASGSDINDYPISWVRQAPGKGLEWIGFINSGGSTWYASWVKGRFTISRTSTTVDLKMTSLTTDDTATYFCARGYSTYYGDFNIWGPGTLVTISSGGGGSGGGGSGGGGSELVMTQTPSSTSGAVGGTVTINCQASQSIDSNLAWFQQKPGQPPTLLIYRASNLASGVPSRFSGSRSGTEYTLTISGVQREDAATYYCLGGVGNVSYRTSFGGGTEVVVKESKYGPPCPPCPGQPREPQVYTLPPSQEEMTKNQVSLTCLVKGFYPSDIAVEWESNGQPENNYKTTPPVLDSDGSFFLYSRLTVDKSRWQEGNVFSCSVMHEALHNHYTQKSLSLSLGKMFWVLVVVGGVLACYSLLVTVAFIIFWVKRGRKKLLYIFKQPFMRPVQTTQEEDGCSCRFPEEEEGGCELRVKFSRSADAPAYQQGQNQLYNELNLGRREEYDVLDKRRGRDPEMGGKPRRKNPQEGLYNELQKDKMAEAYSEIGMKGERRRGKGHDGLYQGLSTATKDTYDALHMQALPPRLEGGGEGRGSLLTCGDVEENPGPRMLLLVTSLLLCELPHPAFLLIPRKVCNGIGIGEFKDSLSINATNIKHFKNCTSISGDLHILPVAFRGDSFTHTPPLDPQELDILKTVKEITGFLLIQAWPENRTDLHAFENLEIIRGRTKQHGQFSLAVVSLNITSLGLRSLKEISDGDVIISGNKNLCYANTINWKKLFGTSGQKTKIISNRGENSCKATGQVCHALCSPEGCWGPEPRDCVSCRNVSRGRECVDKCNLLEGEPREFVENSECIQCHPECLPQAMNITCTGRGPDNCIQCAHYIDGPHCVKTCPAGVMGENNTLVWKYADAGHVCHLCHPNCTYGCTGPGLEGCPTNGPKIPSIATGMVGALLLLLVVALGIGLFM

SEQ ID NO: 47 - DNA, 9685 bp, Artificial Sequence
  Synthetic
gttagaccagatctgagcctgggagctctctggctaactagggaacccactgcttaagcctcaataaagcttgccttgagtgcttcaagtagtgtgtgcccgtctgttgtgtgactctggtaactagagatccctcagacccttttagtcagtgtggaaaatctctagcagtggcgcccgaacagggacttgaaagcgaaagggaaaccagaggagctctctcgacgcaggactcggcttgctgaagcgcgcacggcaagaggcgaggggcggcgactggtgagtacgccaaaaattttgactagcggaggctagaaggagagagatgggtgcgagagcgtcagtattaagcgggggagaattagatcgatgggaaaaaattcggttaaggccagggggaaagaaaaaatataaattaaaacatatagtatgggcaagcagggagctagaacgattcgcagttaatcctggcctgttagaaacatcagaaggctgtagacaaatactgggacagctacaaccatcccttcagacaggatcagaagaacttagatcattatataatacagtagcaaccctctattgtgtgcatcaaaggatagagataaaagacaccaaggaagctttagacaagatagaggaagagcaaaacaaaagtaagaaaaaagcacagcaagcagcagctgacacaggacacagcaatcaggtcagccaaaattaccctatagtgcagaacatccaggggcaaatggtacatcaggccatatcacctagaactttaaatgcatgggtaaaagtagtagaagagaaggctttcagcccagaagtgatacccatgttttcagcattatcagaaggagccaccccacaagatttaaacaccatgctaaacacagtggggggacatcaagcagccatgcaaatgttaaaagagaccatcaatgaggaagctgcaggcaaagagaagagtggtgcagagagaaaaaagagcagtgggaataggagctttgttccttgggttcttgggagcagcaggaagcactatgggcgcagcgtcaatgacgctgacggtacaggccagacaattattgtctggtatagtgcagcagcagaacaatttgctgagggctattgaggcgcaacagcatctgttgcaactcacagtctggggcatcaagcagctccaggcaagaatcctggctgtggaaagatacctaaaggatcaacagctcctggggatttggggttgctctggaaaactcatttgcaccactgctgtgccttggatctacaaatggcagtattcatccacaattttaaaagaaaaggggggattggggggtacagtgcaggggaaagaatagtagacataatagcaacagacatacaaactaaagaattacaaaaacaaattacaaaaattcaaaattttcgggtttattacagggacagcagagatccagtttggggatcaattgcatgaagaatctgcttagggttaggcgttttgcgctgcttcgcgaggatctgcgatcgctccggtgcccgtcagtgggcagagcgcacatcgcccacagtccccgagaagttggggggaggggtcggcaattgaaccggtgcctagagaaggtggcgcggggtaaactgggaaagtgatgtcgtgtactggctccgcctttttcccgagggtgggggagaaccgtatataagtgcagtagtcgccgtgaacgttctttttcgcaacgggtttgccgccagaacacagctgaagcttcgaggggctcgcatctctccttcacgcgcccgccgccctacctgaggccgccatccacgccggttgagtcgcgttctgccgcctcccgcctgtggtgcctcctgaactgcgtccgccgtctaggtaagtttaaagctcaggtcgagaccgggcctttgtccggcgctcccttggagcctacctagactcagccggctctccacgctttgcctgaccctgcttgctcaactctacgtctttgtttcgttttctgttctgcgccgttacagatccaagctgtgaccggcgcctacggctagcgaattcgccaccatgctgctgctggtgacaagcctgctgctgtgcgagctgccccaccccgcctttctgctgatcccccagagcgtgaaagagtccgagggcgacctggtcacaccagccggcaacctgaccctgacctgtaccgccagcggcagcgacatcaacgactaccccatctcttgggtccgccaggctcctggcaagggactggaatggatcggcttcatcaacagcggcggcagcacttggtacgccagctgggtcaaaggccggttcaccatcagccggaccagcaccaccgtggacctgaagatgacaagcctgaccaccgacgacaccgccacctacttttgcgccagaggctacagcacctactacggcgacttcaacatctggggccctggcaccctggtcacaatctctagcggcggaggcggcagcggaggtggaggaagtggcggcggaggatccgagctggtcatgacccagacccccagcagcacatctggcgccgtgggcggcaccgtgaccatcaattgccaggccagccagagcatcgacagcaacctggcctggttccagcagaagcccggccagccccccaccctgctgatctacagagcctccaacctggccagcggcgtgccaagcagattcagcggcagcagatctggcaccgagtacaccctgaccatctccggcgtgcagagagaggacgccgctacctattactgcctgggcggcgtgggcaacgtgtcctacagaaccagcttcggcggaggtactgaggtggtcgtcaaatacggaccgccctgccccccttgccctggccagcctcgcgagccccaggtgtacaccctgcctccctcccaggaagagatgaccaagaaccaggtgtccctgacctgcctggtgaagggcttctaccccagcgacatcgccgtggagtgggagagcaacggccagcctgagaacaactacaagaccacccctcccgtgctggacagcgacggcagcttcttcctgtacagccggctgaccgtggacaagagccggtggcaggaaggcaacgtctttagctgcagcgtgatgcacgaggccctgcacaaccactacacccagaagagcctgagcctgtccctgggcaagatgttctgggtgctggtggtggtgggcggggtgctggcctgctacagcctgctggtgacagtggccttcatcatcttttgggtgaaacggggcagaaagaaactcctgtatatattcaaacaaccatttatgagaccagtacaaactactcaagaggaagatggctgtagctgccgatttccagaagaagaagaaggaggatgtgaactgcgggtgaagttcagcagaagcgccgacgcccctgcctaccagcagggccagaatcagctgtacaacgagctgaacctgggcagaagggaagagtacgacgtcctggataagcggagaggccgggaccctgagatgggcggcaagcctcggcggaagaacccccaggaaggcctgtataacgaactgcagaaagacaagatggccgaggcctacagcgagatcggcatgaagggcgagcggaggcggggcaagggccacgacggcctgtatcagggcctgtccaccgccaccaaggatacctacgacgccctgcacatgcaggccctgcccccaaggctcgagggcggcggagagggcagaggaagtcttctaacatgcggtgacgtggaggagaatcccggccctaggatgcttctcctggtgacaagccttctgctctgtgagttaccacacccagcattcctcctgatcccacgcaaagtgtgtaacggaataggtattggtgaatttaaagactcactctccataaatgctacgaatattaaacacttcaaaaactgcacctccatcagtggcgatctccacatcctgccggtggcatttaggggtgactccttcacacatactcctcctctggatccacaggaactggatattctgaaaaccgtaaaggaaatcacagggtttttgctgattcaggcttggcctgaaaacaggacggacctccatgcctttgagaacctagaaatcatacgcggcaggaccaagcaacatggtcagttttctcttgcagtcgtcagcctgaacataacatccttgggattacgctccctcaaggagataagtgatggagatgtgataatttcaggaaacaaaaatttgtgctatgcaaatacaataaactggaaaaaactgtttgggacctccggtcagaaaaccaaaattataagcaacagaggtgaaaacagctgcaaggccacaggccaggtctgccatgccttgtgctcccccgagggctgctggggcccggagcccagggactgcgtctcttgccggaatgtcagccgaggcagggaatgcgtggacaagtgcaaccttctggagggtgagccaagggagtttgtggagaactctgagtgcatacagtgccacccagagtgcctgcctcaggccatgaacatcacctgcacaggacggggaccagacaactgtatccagtgtgcccactacattgacggcccccactgcgtcaagacctgcccggcaggagtcatgggagaaaacaacaccctggtctggaagtacgcagacgccggccatgtgtgccacctgtgccatccaaactgcacctacggatgcactgggccaggtcttgaaggctgtccaacgaatgggcctaagatcccgtccatcgccactgggatggtgggggccctcctcttgctgctggtggtggccctggggatcggcctcttcatgtgagcggccgctctagacccgggctgcaggaattcgatatcaagcttatcgataatcaacctctggattacaaaatttgtgaaagattgactggtattcttaactatgttgctccttttacgctatgtggatacgctgctttaatgcctttgtatcatgctattgcttcccgtatggctttcattttctcctccttgtataaatcctggttgctgtctctttatgaggagttgtggcccgttgtcaggcaacgtggcgtggtgtgcactgtgtttgctgacgcaacccccactggttggggcattgccaccacctgtcagctcctttccgggactttcgctttccccctccctattgccacggcggaactcatcgccgcctgccttgcccgctgctggacaggggctcggctgttgggcactgacaattccgtggtgttgtcggggaaatcatcgtcctttccttggctgctcgcctgtgttgccacctggattctgcgcgggacgtccttctgctacgtcccttcggccctcaatccagcggaccttccttcccgcggcctgctgccggctctgcggcctcttccgcgtcttcgccttcgccctcagacgagtcggatctccctttgggccgcctccccgcatcgataccgtcgactagccgtacctttaagaccaatgacttacaaggcagctgtagatcttagccactttttaaaagaaaaggggggactggaagggctaattcactcccaaagaagacaagatctgctttttgcctgtactgggtctctctggttagaccagatctgagcctgggagctctctggctaactagggaacccactgcttaagcctcaataaagcttgccttgagtgcttcaagtagtgtgtgcccgtctgttgtgtgactctggtaactagagatccctcagacccttttagtcagtgtggaaaatctctagcagaattcgatatcaagcttatcgataccgtcgacctcgagggggggcccggtacccaattcgccctatagtgagtcgtattacaattcactggccgtcgttttacaacgtcgtgactgggaaaaccctggcgttacccaacttaatcgccttgcagcacatccccctttcgccagctggcgtaatagcgaagaggcccgcaccgatcgcccttcccaacagttgcgcagcctgaatggcgaatggaaattgtaagcgttaatattttgttaaaattcgcgttaaatttttgttaaatcagctcattttttaaccaataggccgaaatcggcaaaatcccttataaatcaaaagaatagaccgagatagggttgagtgttgttccagtttggaacaagagtccactattaaagaacgtggactccaacgtcaaagggcgaaaaaccgtctatcagggcgatggcccactacgtgaaccatcaccctaatcaagttttttggggtcgaggtgccgtaaagcactaaatcggaaccctaaagggagcccccgatttagagcttgacggggaaagccggcgaacgtggcgagaaaggaagggaagaaagcgaaaggagcgggcgctagggcgctggcaagtgtagcggtcacgctgcgcgtaaccaccacacccgccgcgcttaatgcgccgctacagggcgcgtcaggtggcacttttcggggaaatgtgcgcggaacccctatttgtttatttttctaaatacattcaaatatgtatccgctcatgagacaataaccctgataaatgcttcaataatattgaaaaaggaagagtatgagtattcaacatttccgtgtcgcccttattcccttttttgcggcattttgccttcctgtttttgctcacccagaaacgctggtgaaagtaaaagatgctgaagatcagttgggtgcacgagtgggttacatcgaactggatctcaacagcggtaagatccttgagagttttcgccccgaagaacgttttccaatgatgagcacttttaaagttctgctatgtggcgcggtattatcccgtattgacgccgggcaagagcaactcggtcgccgcatacactattctcagaatgacttggttgagtactcaccagtcacagaaaagcatcttacggatggcatgacagtaagagaattatgcagtgctgccataaccatgagtgataacactgcggccaacttacttctgacaacgatcggaggaccgaaggagctaaccgcttttttgcacaacatgggggatcatgtaactcgccttgatcgttgggaaccggagctgaatgaagccataccaaacgacgagcgtgacaccacgatgcctgtagcaatggcaacaacgttgcgcaaactattaactggcgaactacttactctagcttcccggcaacaattaatagactggatggaggcggataaagttgcaggaccacttctgcgctcggcccttccggctggctggtttattgctgataaatctggagccggtgagcgtgggtctcgcggtatcattgcagcactggggccagatggtaagccctcccgtatcgtagttatctacacgacggggagtcaggcaactatggatgaacgaaatagacagatcgctgagataggtgcctcactgattaagcattggtaactgtcagaccaagtttactcatatatactttagattgatttaaaacttcatttttaatttaaaaggatctaggtgaagatcctttttgataatctcatgaccaaaatcccttaacgtgagttttcgttccactgagcgtcagaccccgtagaaaagatcaaaggatcttcttgagatcctttttttctgcgcgtaatctgctgcttgcaaacaaaaaaaccaccgctaccagcggtggtttgtttgccggatcaagagctaccaactctttttccgaaggtaactggcttcagcagagcgcagataccaaatactgttcttctagtgtagccgtagttaggccaccacttcaagaactctgtagcaccgcctacatacctcgctctgctaatcctgttaccagtggctgctgccagtggcgataagtcgtgtcttaccgggttggactcaagacgatagttaccggataaggcgcagcggtcgggctgaacggggggttcgtgcacacagcccagcttggagcgaacgacctacaccgaactgagatacctacagcgtgagctatgagaaagcgccacgcttcccgaagggagaaaggcggacaggtatccggtaagcggcagggtcggaacaggagagcgcacgagggagcttccagggggaaacgcctggtatctttatagtcctgtcgggtttcgccacctctgacttgagcgtcgatttttgtgatgctcgtcaggggggcggagcctatggaaaaacgccagcaacgcggcctttttacggttcctggccttttgctggccttttgctcacatgttctttcctgcgttatcccctgattctgtggataaccgtattaccgcctttgagtgagctgataccgctcgccgcagccgaacgaccgagcgcagcgagtcagtgagcgaggaagcggaagagcgcccaatacgcaaaccgcctctccccgcgcgttggccgattcattaatgcagctggcacgacaggtttcccgactggaaagcgggcagtgagcgcaacgcaattaatgtgagttagctcactcattaggcaccccaggctttacactttatgcttccggctcgtatgttgtgtggaattgtgagcggataacaatttcacacaggaaacagctatgaccatgattacgccaagctcgaaattaaccctcactaaagggaacaaaagctggagctccaccgcggtggcggcctcgaggtcgagatccggtcgaccagcaaccatagtcccgcccctaactccgcccatcccgcccctaactccgcccagttccgcccattctccgccccatggctgactaattttttttatttatgcagaggccgaggccgcctcggcctctgagctattccagaagtagtgaggaggcttttttggaggcctaggcttttgcaaaaagcttcgacggtatcgattggctcatgtccaacattaccgccatgttgacattgattattgactagttattaatagtaatcaattacggggtcattagttcatagcccatatatggagttccgcgttacataacttacggtaaatggcccgcctggctgaccgcccaacgacccccgcccattgacgtcaataatgacgtatgttcccatagtaacgccaatagggactttccattgacgtcaatgggtggagtatttacggtaaactgcccacttggcagtacatcaagtgtatcatatgccaagtacgccccctattgacgtcaatgacggtaaatggcccgcctggcattatgcccagtacatgaccttatgggactttcctacttggcagtacatctacgtattagtcatcgctattaccatggtgatgcggttttggcagtacatcaatgggcgtggatagcggtttgactcacggggatttccaagtctccaccccattgacgtcaatgggagtttgttttggcaccaaaatcaacgggactttccaaaatgtcgtaacaactccgccccattgacgcaaatgggcggtaggcgtgtacggaattcggagtggcgagccctcagatcctgcatataagcagctgctttttgcctgtactgggtctctctg

SEQ ID NO: 48 - protein, 838 aa, Artificial Sequence
  Synthetic
MLLLVTSLLLCELPHPAFLLIPQSVKESEGDLVTPAGNLTLTCTASGSDINDYPISWVRQAPGKGLEWIGFINSGGSTWYASWVKGRFTISRTSTTVDLKMTSLTTDDTATYFCARGYSTYYGDFNIWGPGTLVTISSGGGGSGGGGSGGGGSELVMTQTPSSTSGAVGGTVTINCQASQSIDSNLAWFQQKPGQPPTLLIYRASNLASGVPSRFSGSRSGTEYTLTISGVQREDAATYYCLGGVGNVSYRTSFGGGTEVVVKESKYGPPCPPCPMFWVLVVVGGVLACYSLLVTVAFIIFWVKRGRKKLLYIFKQPFMRPVQTTQEEDGCSCRFPEEEEGGCELRVKFSRSADAPAYQQGQNQLYNELNLGRREEYDVLDKRRGRDPEMGGKPRRKNPQEGLYNELQKDKMAEAYSEIGMKGERRRGKGHDGLYQGLSTATKDTYDALHMQALPPRLEGGGEGRGSLLTCGDVEENPGPRMLLLVTSLLLCELPHPAFLLIPRKVCNGIGIGEFKDSLSINATNIKHFKNCTSISGDLHILPVAFRGDSFTHTPPLDPQELDILKTVKEITGFLLIQAWPENRTDLHAFENLEIIRGRTKQHGQFSLAVVSLNITSLGLRSLKEISDGDVIISGNKNLCYANTINWKKLFGTSGQKTKIISNRGENSCKATGQVCHALCSPEGCWGPEPRDCVSCRNVSRGRECVDKCNLLEGEPREFVENSECIQCHPECLPQAMNITCTGRGPDNCIQCAHYIDGPHCVKTCPAGVMGENNTLVWKYADAGHVCHLCHPNCTYGCTGPGLEGCPTNGPKIPSIATGMVGALLLLLVVALGIGLFM

SEQ ID NO: 49 - protein, 119 aa, Artificial Sequence
  Synthetic
ESKYGPPCPPCPGQPREPQVYTLPPSQEEMTKNQVSLTCLVKGFYPSDIAVEWESNGQPENNYKTTPPVLDSDGSFFLYSRLTVDKSRWQEGNVFSCSVMHEALHNHYTQKSLSLSLGK

SEQ ID NO: 50 - protein, 229 aa, Artificial Sequence
  Synthetic
ESKYGPPCPPCPAPEFLGGPSVFLFPPKPKDTLMISRTPEVTCVVVDVSQEDPEVQFNWYVDGVEVHNAKTKPREEQFNSTYRVVSVLTVLHQDWLNGKEYKCKVSNKGLPSSIEKTISKAKGQPREPQVYTLPPSQEEMTKNQVSLTCLVKGFYPSDIAVEWESNGQPENNYKTTPPVLDSDGSFFLYSRLTVDKSRWQEGNVFSCSVMHEALHNHYTQKSLSLSLGK

SEQ ID NO: 51 - protein, 9 aa, Artificial Sequence
  Synthetic
YGPPCPPCP

SEQ ID NO: 52 - protein, 10 aa, Artificial Sequence
  Synthetic
KYGPPCPPCP

SEQ ID NO: 53 - protein, 14 aa, Artificial Sequence
  Synthetic
EVVVKYGPPCPPCP

SEQ ID NO: 54 - DNA, 2529 bp, Artificial Sequence
  Synthetic
atgcttctcctggtgacaagccttctgctctgtgagttaccacacccagcattcctcctgatcccagatatccagatgacccagtccccgagctccctgtccgcctctgtgggcgatagggtcaccatcacctgccgtgccagtcaggatgtgaatactgctgtagcctggtatcaacagaaaccaggaaaagctccgaaactactgatttactcggcatccttcctctactctggagtcccttctcgcttctctggttccagatctgggacggatttcactctgaccatcagcagtctgcagccggaagacttcgcaacttattactgtcagcaacattatactactcctcccacgttcggacagggtaccaaggtggagatcaaaggcagtactagcggcggtggctccgggggcggatccggtgggggcggcagcagcgaggttcagctggtggagtctggcggtggcctggtgcagccagggggctcactccgtttgtcctgtgcagcttctggcttcaacattaaagacacctatatacactgggtgcgtcaggccccgggtaagggcctggaatgggttgcaaggatttatcctacgaatggttatactagatatgccgatagcgtcaagggccgtttcactataagcgcagacacatccaaaaacacagcctacctgcagatgaacagcctgcgtgctgaggacactgccgtctattattgttctagatggggaggggacggcttctatgctatggactactggggtcaaggaaccctggtcaccgtctcgagtgagagcaagtacggaccgccctgccccccttgccctatgttctgggtgctggtggtggtcggaggcgtgctggcctgctacagcctgctggtcaccgtggccttcatcatcttttgggtgaaacggggcagaaagaaactcctgtatatattcaaacaaccatttatgagaccagtacaaactactcaagaggaagatggctgtagctgccgatttccagaagaagaagaaggaggatgtgaactgcgggtgaagttcagcagaagcgccgacgcccctgcctaccagcagggccagaatcagctgtacaacgagctgaacctgggcagaagggaagagtacgacgtcctggataagcggagaggccgggaccctgagatgggcggcaagcctcggcggaagaacccccaggaaggcctgtataacgaactgcagaaagacaagatggccgaggcctacagcgagatcggcatgaagggcgagcggaggcggggcaagggccacgacggcctgtatcagggcctgtccaccgccaccaaggatacctacgacgccctgcacatgcaggccctgcccccaaggctcgagggcggcggagagggcagaggaagtcttctaacatgcggtgacgtggaggagaatcccggccctaggatgcttctcctggtgacaagccttctgctctgtgagttaccacacccagcattcctcctgatcccacgcaaagtgtgtaacggaataggtattggtgaatttaaagactcactctccataaatgctacgaatattaaacacttcaaaaactgcacctccatcagtggcgatctccacatcctgccggtggcatttaggggtgactccttcacacatactcctcctctggatccacaggaactggatattctgaaaaccgtaaaggaaatcacagggtttttgctgattcaggcttggcctgaaaacaggacggacctccatgcctttgagaacctagaaatcatacgcggcaggaccaagcaacatggtcagttttctcttgcagtcgtcagcctgaacataacatccttgggattacgctccctcaaggagataagtgatggagatgtgataatttcaggaaacaaaaatttgtgctatgcaaatacaataaactggaaaaaactgtttgggacctccggtcagaaaaccaaaattataagcaacagaggtgaaaacagctgcaaggccacaggccaggtctgccatgccttgtgctcccccgagggctgctggggcccggagcccagggactgcgtctcttgccggaatgtcagccgaggcagggaatgcgtggacaagtgcaaccttctggagggtgagccaagggagtttgtggagaactctgagtgcatacagtgccacccagagtgcctgcctcaggccatgaacatcacctgcacaggacggggaccagacaactgtatccagtgtgcccactacattgacggcccccactgcgtcaagacctgcccggcaggagtcatgggagaaaacaacaccctggtctggaagtacgcagacgccggccatgtgtgccacctgtgccatccaaactgcacctacggatgcactgggccaggtcttgaaggctgtccaacgaatgggcctaagatcccgtccatcgccactgggatggtgggggccctcctcttgctgctggtggtggccctggggatcggcctcttcatgtga

SEQ ID NO: 55 - DNA, 2850 bp, Artificial Sequence
  Synthetic
atgcttctcctggtgacaagccttctgctctgtgagttaccacacccagcattcctcctgatcccagatatccagatgacccagtccccgagctccctgtccgcctctgtgggcgatagggtcaccatcacctgccgtgccagtcaggatgtgaatactgctgtagcctggtatcaacagaaaccaggaaaagctccgaaactactgatttactcggcatccttcctctactctggagtcccttctcgcttctctggttccagatctgggacggatttcactctgaccatcagcagtctgcagccggaagacttcgcaacttattactgtcagcaacattatactactcctcccacgttcggacagggtaccaaggtggagatcaaaggcagtactagcggcggtggctccgggggcggatccggtgggggcggcagcagcgaggttcagctggtggagtctggcggtggcctggtgcagccagggggctcactccgtttgtcctgtgcagcttctggcttcaacattaaagacacctatatacactgggtgcgtcaggccccgggtaagggcctggaatgggttgcaaggatttatcctacgaatggttatactagatatgccgatagcgtcaagggccgtttcactataagcgcagacacatccaaaaacacagcctacctgcagatgaacagcctgcgtgctgaggacactgccgtctattattgttctagatggggaggggacggcttctatgctatggactactggggtcaaggaaccctggtcaccgtctcgagtgagagcaagtacggaccgccctgccccccttgccctggccagcctagagaaccccaggtgtacaccctgcctcccagccaggaagagatgaccaagaaccaggtgtccctgacctgcctggtcaaaggcttctaccccagcgatatcgccgtggaatgggagagcaacggccagcccgagaacaactacaagaccaccccccctgtgctggacagcgacggcagcttcttcctgtactcccggctgaccgtggacaagagccggtggcaggaaggcaacgtcttcagctgcagcgtgatgcacgaggccctgcacaaccactacacccagaagtccctgagcctgagcctgggcaagatgttctgggtgctggtggtggtcggaggcgtgctggcctgctacagcctgctggtcaccgtggccttcatcatcttttgggtgaaacggggcagaaagaaactcctgtatatattcaaacaaccatttatgagaccagtacaaactactcaagaggaagatggctgtagctgccgatttccagaagaagaagaaggaggatgtgaactgcgggtgaagttcagcagaagcgccgacgcccctgcctaccagcagggccagaatcagctgtacaacgagctgaacctgggcagaagggaagagtacgacgtcctggataagcggagaggccgggaccctgagatgggcggcaagcctcggcggaagaacccccaggaaggcctgtataacgaactgcagaaagacaagatggccgaggcctacagcgagatcggcatgaagggcgagcggaggcggggcaagggccacgacggcctgtatcagggcctgtccaccgccaccaaggatacctacgacgccctgcacatgcaggccctgcccccaaggctcgagggcggcggagagggcagaggaagtcttctaacatgcggtgacgtggaggagaatcccggccctaggatgcttctcctggtgacaagccttctgctctgtgagttaccacacccagcattcctcctgatcccacgcaaagtgtgtaacggaataggtattggtgaatttaaagactcactctccataaatgctacgaatattaaacacttcaaaaactgcacctccatcagtggcgatctccacatcctgccggtggcatttaggggtgactccttcacacatactcctcctctggatccacaggaactggatattctgaaaaccgtaaaggaaatcacagggtttttgctgattcaggcttggcctgaaaacaggacggacctccatgcctttgagaacctagaaatcatacgcggcaggaccaagcaacatggtcagttttctcttgcagtcgtcagcctgaacataacatccttgggattacgctccctcaaggagataagtgatggagatgtgataatttcaggaaacaaaaatttgtgctatgcaaatacaataaactggaaaaaactgtttgggacctccggtcagaaaaccaaaattataagcaacagaggtgaaaacagctgcaaggccacaggccaggtctgccatgccttgtgctcccccgagggctgctggggcccggagcccagggactgcgtctcttgccggaatgtcagccgaggcagggaatgcgtggacaagtgcaaccttctggagggtgagccaagggagtttgtggagaactctgagtgcatacagtgccacccagagtgcctgcctcaggccatgaacatcacctgcacaggacggggaccagacaactgtatccagtgtgcccactacattgacggcccccactgcgtcaagacctgcccggcaggagtcatgggagaaaacaacaccctggtctggaagtacgcagacgccggccatgtgtgccacctgtgccatccaaactgcacctacggatgcactgggccaggtcttgaaggctgtccaacgaatgggcctaagatcccgtccatcgccactgggatggtgggggccctcctcttgctgctggtggtggccctggggatcggcctcttcatgtga

SEQ ID NO: 56 - DNA, 3180 bp, Artificial Sequence
  Synthetic
atgcttctcctggtgacaagccttctgctctgtgagttaccacacccagcattcctcctgatcccagatatccagatgacccagtccccgagctccctgtccgcctctgtgggcgatagggtcaccatcacctgccgtgccagtcaggatgtgaatactgctgtagcctggtatcaacagaaaccaggaaaagctccgaaactactgatttactcggcatccttcctctactctggagtcccttctcgcttctctggttccagatctgggacggatttcactctgaccatcagcagtctgcagccggaagacttcgcaacttattactgtcagcaacattatactactcctcccacgttcggacagggtaccaaggtggagatcaaaggcagtactagcggcggtggctccgggggcggatccggtgggggcggcagcagcgaggttcagctggtggagtctggcggtggcctggtgcagccagggggctcactccgtttgtcctgtgcagcttctggcttcaacattaaagacacctatatacactgggtgcgtcaggccccgggtaagggcctggaatgggttgcaaggatttatcctacgaatggttatactagatatgccgatagcgtcaagggccgtttcactataagcgcagacacatccaaaaacacagcctacctgcagatgaacagcctgcgtgctgaggacactgccgtctattattgttctagatggggaggggacggcttctatgctatggactactggggtcaaggaaccctggtcaccgtctcgagtgagagcaagtacggaccgccctgccccccttgccctgcccccgagttcctgggcggacccagcgtgttcctgttcccccccaagcccaaggacaccctgatgatcagccggacccccgaggtgacctgcgtggtggtggacgtgagccaggaagatcccgaggtccagttcaattggtacgtggacggcgtggaagtgcacaacgccaagaccaagcccagagaggaacagttcaacagcacctaccgggtggtgtctgtgctgaccgtgctgcaccaggactggctgaacggcaaagaatacaagtgcaaggtgtccaacaagggcctgcccagcagcatcgaaaagaccatcagcaaggccaagggccagcctcgcgagccccaggtgtacaccctgcctccctcccaggaagagatgaccaagaaccaggtgtccctgacctgcctggtgaagggcttctaccccagcgacatcgccgtggagtgggagagcaacggccagcctgagaacaactacaagaccacccctcccgtgctggacagcgacggcagcttcttcctgtacagccggctgaccgtggacaagagccggtggcaggaaggcaacgtctttagctgcagcgtgatgcacgaggccctgcacaaccactacacccagaagagcctgagcctgtccctgggcaagatgttctgggtgctggtggtggtgggcggggtgctggcctgctacagcctgctggtgacagtggccttcatcatcttttgggtgaaacggggcagaaagaaactcctgtatatattcaaacaaccatttatgagaccagtacaaactactcaagaggaagatggctgtagctgccgatttccagaagaagaagaaggaggatgtgaactgcgggtgaagttcagcagaagcgccgacgcccctgcctaccagcagggccagaatcagctgtacaacgagctgaacctgggcagaagggaagagtacgacgtcctggataagcggagaggccgggaccctgagatgggcggcaagcctcggcggaagaacccccaggaaggcctgtataacgaactgcagaaagacaagatggccgaggcctacagcgagatcggcatgaagggcgagcggaggcggggcaagggccacgacggcctgtatcagggcctgtccaccgccaccaaggatacctacgacgccctgcacatgcaggccctgcccccaaggctcgagggcggcggagagggcagaggaagtcttctaacatgcggtgacgtggaggagaatcccggccctaggatgcttctcctggtgacaagccttctgctctgtgagttaccacacccagcattcctcctgatcccacgcaaagtgtgtaacggaataggtattggtgaatttaaagactcactctccataaatgctacgaatattaaacacttcaaaaactgcacctccatcagtggcgatctccacatcctgccggtggcatttaggggtgactccttcacacatactcctcctctggatccacaggaactggatattctgaaaaccgtaaaggaaatcacagggtttttgctgattcaggcttggcctgaaaacaggacggacctccatgcctttgagaacctagaaatcatacgcggcaggaccaagcaacatggtcagttttctcttgcagtcgtcagcctgaacataacatccttgggattacgctccctcaaggagataagtgatggagatgtgataatttcaggaaacaaaaatttgtgctatgcaaatacaataaactggaaaaaactgtttgggacctccggtcagaaaaccaaaattataagcaacagaggtgaaaacagctgcaaggccacaggccaggtctgccatgccttgtgctcccccgagggctgctggggcccggagcccagggactgcgtctcttgccggaatgtcagccgaggcagggaatgcgtggacaagtgcaaccttctggagggtgagccaagggagtttgtggagaactctgagtgcatacagtgccacccagagtgcctgcctcaggccatgaacatcacctgcacaggacggggaccagacaactgtatccagtgtgcccactacattgacggcccccactgcgtcaagacctgcccggcaggagtcatgggagaaaacaacaccctggtctggaagtacgcagacgccggccatgtgtgccacctgtgccatccaaactgcacctacggatgcactgggccaggtcttgaaggctgtccaacgaatgggcctaagatcccgtccatcgccactgggatggtgggggccctcctcttgctgctggtggtggccctggggatcggcctcttcatgtga